European Patent Specification EP 4 003 397 B1, published February 26, 2025. Title: TREATMENT OF CYSTIC FIBROSIS BY DELIVERY OF NEBULIZED mRNA ENCODING CFTR. Applicant: Translate Bio, Inc. The sequence listing filed with the application follows.

SEQUENCE LISTING (30 sequences)

SEQ ID NO: 1 - RNA, 4443 nt, Artificial Sequence
  Synthetic polynucleotide
augcaacgcucuccucuugaaaaggccucggugguguccaagcucuucuucucguggacuagacccauccugagaaagggguacagacagcgcuuggagcuguccgauaucuaucaaaucccuuccguggacuccgcggacaaccuguccgagaagcucgagagagaaugggacagagaacucgccucaaagaagaacccgaagcugauuaaugcgcuuaggcggugcuuuuucuggcgguucauguucuacggcaucuuccucuaccugggagaggucaccaaggccgugcagccccuguugcugggacggauuauugccuccuacgaccccgacaacaaggaagaaagaagcaucgcuaucuacuugggcaucggucugugccugcuuuucaucguccggacccucuuguugcauccugcuauuuucggccugcaucacauuggcaugcagaugagaauugccauguuuucccugaucuacaagaaaacucugaagcucucgagccgcgugcuugacaagauuuccaucggccagcucgugucccugcucuccaacaaucugaacaaguucgacgagggccucgcccuggcccacuucguguggaucgccccucugcaaguggcgcuucugaugggccugaucugggagcugcugcaagccucggcauucugugggcuuggauuccugaucgugcuggcacuguuccaggccggacuggggcggaugaugaugaaguacagggaccagagagccggaaagauuuccgaacggcuggugaucacuucggaaaugaucgaaaacauccagucagugaaggccuacugcugggaagaggccauggaaaagaugauugaaaaccuccggcaaaccgagcugaagcugacccgcaaggccgcuuacgugcgcuauuucaacucguccgcuuucuucuucuccggguucuucgugguguuucucuccgugcuccccuacgcccugauuaagggaaucauccucaggaagaucuucaccaccauuuccuucuguaucgugcuccgcauggccgugacccggcaguucccaugggccgugcagacuugguacgacucccugggagccauuaacaagauccaggacuuccuucaaaagcaggaguacaagacccucgaguacaaccugacuacuaccgaggucgugauggaaaacgucaccgccuuuugggaggagggauuuggcgaacuguucgagaaggccaagcagaacaacaacaaccgcaagaccucgaacggugacgacucccucuucuuuucaaacuucagccugcucgggacgcccgugcugaaggacauuaacuucaagaucgaaagaggacagcuccuggcgguggccggaucgaccggagccggaaagacuucccugcugauggugaucaugggagagcuugaaccuagcgagggaaagaucaagcacuccggccgcaucagcuucuguagccaguuuuccuggaucaugcccggaaccauuaaggaaaacaucaucuucggcguguccuacgaugaauaccgcuaccgguccgugaucaaagccugccagcuggaagaggauauuucaaaguucgcggagaaagauaacaucgugcugggcgaaggggguauuaccuugucggggggccagcgggcuagaaucucgcuggccagagccguguauaaggacgccgaccuguaucuccuggacucccccuucggauaccuggacguccugaccgaaaaggagaucuucgaaucgugcgugugcaagcugauggcuaacaagacucgcauccucgugaccuccaaaauggagcaccugaagaaggcagacaagauucugauucugcaugagggguccuccuacuuuuacggcaccuucucggaguugcagaacuugcagcccgacuucucaucgaagcugauggguugcgacagcuucgaccaguucuccgccgaaagaaggaacucgauccugacggaaaccuugcaccgcuucucuuuggaaggcgacgccccugugucauggaccgagacuaagaagcagagcuucaagcagaccggggaauucggcgaaaagaggaagaacagcaucuugaaccccauuaacuccauccgcaaguucucaaucgugcaaaagacgccacugcagaugaacggcauugaggaggacuccgacgaaccccuugagaggcgccugucccuggugccggacagcgagcagggagaagccauccugccucggauuuccgugaucuccacugguccgacgcuccaagcccggcggcggcaguccgugcugaaccugaugacccacagcgugaaccagggccaaaacauucaccgcaagacuaccgcauccacccggaaagugucccuggcaccucaagcgaaucuuaccgagcucgacaucuacucccggagacugucgcaggaaaccgggcucgaaauuuccgaagaaaucaacgaggaggaucugaaagagugcuucuucgacgauauggagucgauacccgccgugacgacuuggaacacuuaucugcgguacaucacugugcacaagucauugaucuucgugcugauuuggugccuggugauuuuccuggccgaggucgcggccucacugguggugcucuggcuguugggaaacacgccucugcaagacaagggaaacuccacgcacucgagaaacaacagcuaugccgugauuaucacuuccaccuccucuuauuacguguucuacaucuacgucggaguggcggauacccugcucgcgauggguuucuucagaggacugccgcugguccacaccuugaucaccgucagcaagauucuucaccacaagauguugcauagcgugcugcaggcccccauguccacccucaacacucugaaggccggaggcauucugaacagauucuccaaggacaucgcuauccuggacgaucuccugccgcuuaccaucuuugacuucauccagcugcugcugaucgugauuggagcaaucgcagugguggcggugcugcagccuuacauuuucguggccacugugccggucauuguggcguucaucaugcugcgggccuacuuccuccaaaccagccagcagcugaagcaacuggaauccgagggacgaucccccaucuucacucaccuugugacgucguugaagggacuguggacccuccgggcuuucggacggcagcccuacuucgaaacccucuuccacaaggcccugaaccuccacaccgccaauugguuccuguaccuguccacccugcggugguuccagaugcgcaucgagaugauuuucgucaucuucuucaucgcggucacauucaucagcauccugacuaccggagagggagagggacgggucggaauaauccugacccucgccaugaacauuaugagcacccugcagugggcagugaacagcucgaucgacguggacagccugaugcgaagcgucagccgcguguucaaguucaucgacaugccuacugagggaaaacccacuaaguccacuaagcccuacaaaaauggccagcugagcaaggucaugaucaucgaaaacucccacgugaagaaggacgauauuuggcccuccggaggucaaaugaccgugaaggaccugaccgcaaaguacaccgagggaggaaacgccauucucgaaaacaucagcuucuccauuucgccgggacagcgggucggccuucucgggcggaccgguuccgggaagucaacucugcugucggcuuuccuccggcugcugaauaccgagggggaaauccaaauugacggcgugucuugggauuccauuacucugcagcaguggcggaaggccuucggcgugaucccccagaagguguucaucuucucggguaccuuccggaagaaccuggauccuuacgagcaguggagcgaccaagaaaucuggaaggucgccgacgaggucggccugcgcuccgugauugaacaauuuccuggaaagcuggacuucgugcucgucgacgggggauguguccugucgcacggacauaagcagcucaugugccucgcacgguccgugcucuccaaggccaagauucugcugcuggacgaaccuucggcccaccuggauccggucaccuaccagaucaucaggaggacccugaagcaggccuuugccgauugcaccgugauucucugcgagcaccgcaucgaggccaugcuggagugccagcaguuccuggucaucgaggagaacaagguccgccaauacgacuccauucaaaagcuccucaacgagcggucgcuguucagacaagcuauuucaccguccgauagagugaagcucuucccgcaucggaacagcucaaagugcaaaucgaagccgcagaucgcagccuugaaggaagagacugaggaagaggugcaggacacccggcuuuaa

SEQ ID NO: 2 - protein, 1480 aa, Homo sapiens
MQRSPLEKASVVSKLFFSWTRPILRKGYRQRLELSDIYQIPSVDSADNLSEKLEREWDRELASKKNPKLINALRRCFFWRFMFYGIFLYLGEVTKAVQPLLLGRIIASYDPDNKEERSIAIYLGIGLCLLFIVRTLLLHPAIFGLHHIGMQMRIAMFSLIYKKTLKLSSRVLDKISIGQLVSLLSNNLNKFDEGLALAHFVWIAPLQVALLMGLIWELLQASAFCGLGFLIVLALFQAGLGRMMMKYRDQRAGKISERLVITSEMIENIQSVKAYCWEEAMEKMIENLRQTELKLTRKAAYVRYFNSSAFFFSGFFVVFLSVLPYALIKGIILRKIFTTISFCIVLRMAVTRQFPWAVQTWYDSLGAINKIQDFLQKQEYKTLEYNLTTTEVVMENVTAFWEEGFGELFEKAKQNNNNRKTSNGDDSLFFSNFSLLGTPVLKDINFKIERGQLLAVAGSTGAGKTSLLMVIMGELEPSEGKIKHSGRISFCSQFSWIMPGTIKENIIFGVSYDEYRYRSVIKACQLEEDISKFAEKDNIVLGEGGITLSGGQRARISLARAVYKDADLYLLDSPFGYLDVLTEKEIFESCVCKLMANKTRILVTSKMEHLKKADKILILHEGSSYFYGTFSELQNLQPDFSSKLMGCDSFDQFSAERRNSILTETLHRFSLEGDAPVSWTETKKQSFKQTGEFGEKRKNSILNPINSIRKFSIVQKTPLQMNGIEEDSDEPLERRLSLVPDSEQGEAILPRISVISTGPTLQARRRQSVLNLMTHSVNQGQNIHRKTTASTRKVSLAPQANLTELDIYSRRLSQETGLEISEEINEEDLKECFFDDMESIPAVTTWNTYLRYITVHKSLIFVLIWCLVIFLAEVAASLVVLWLLGNTPLQDKGNSTHSRNNSYAVIITSTSSYYVFYIYVGVADTLLAMGFFRGLPLVHTLITVSKILHHKMLHSVLQAPMSTLNTLKAGGILNRFSKDIAILDDLLPLTIFDFIQLLLIVIGAIAVVAVLQPYIFVATVPVIVAFIMLRAYFLQTSQQLKQLESEGRSPIFTHLVTSLKGLWTLRAFGRQPYFETLFHKALNLHTANWFLYLSTLRWFQMRIEMIFVIFFIAVTFISILTTGEGEGRVGIILTLAMNIMSTLQWAVNSSIDVDSLMRSVSRVFKFIDMPTEGKPTKSTKPYKNGQLSKVMIIENSHVKKDDIWPSGGQMTVKDLTAKYTEGGNAILENISFSISPGQRVGLLGRTGSGKSTLLSAFLRLLNTEGEIQIDGVSWDSITLQQWRKAFGVIPQKVFIFSGTFRKNLDPYEQWSDQEIWKVADEVGLRSVIEQFPGKLDFVLVDGGCVLSHGHKQLMCLARSVLSKAKILLLDEPSAHLDPVTYQIIRRTLKQAFADCTVILCEHRIEAMLECQQFLVIEENKVRQYDSIQKLLNERSLFRQAISPSDRVKLFPHRNSSKCKSKPQIAALKEETEEEVQDTRL

SEQ ID NO: 3 - RNA, 140 nt, Artificial Sequence
  Synthetic polynucleotide
ggacagaucgccuggagacgccauccacgcuguuuugaccuccauagaagacaccgggaccgauccagccuccgcggccgggaacggugcauuggaacgcggauuccccgugccaagagugacucaccguccuugacacg

SEQ ID NO: 4 - RNA, 105 nt, Artificial Sequence
  Synthetic polynucleotide
cggguggcaucccugugaccccuccccagugccucuccuggcccuggaaguugccacuccagugcccaccagccuuguccuaauaaaauuaaguugcaucaagcu

SEQ ID NO: 5 - RNA, 105 nt, Artificial Sequence
  Synthetic polynucleotide
ggguggcaucccugugaccccuccccagugccucuccuggcccuggaaguugccacuccagugcccaccagccuuguccuaauaaaauuaaguugcaucaaagcu

SEQ ID NO: 6 - RNA, 4688 nt, Artificial Sequence
  Synthetic polynucleotide
ggacagaucgccuggagacgccauccacgcuguuuugaccuccauagaagacaccgggaccgauccagccuccgcggccgggaacggugcauuggaacgcggauuccccgugccaagagugacucaccguccuugacacgaugcaacgcucuccucuugaaaaggccucggugguguccaagcucuucuucucguggacuagacccauccugagaaagggguacagacagcgcuuggagcuguccgauaucuaucaaaucccuuccguggacuccgcggacaaccuguccgagaagcucgagagagaaugggacagagaacucgccucaaagaagaacccgaagcugauuaaugcgcuuaggcggugcuuuuucuggcgguucauguucuacggcaucuuccucuaccugggagaggucaccaaggccgugcagccccuguugcugggacggauuauugccuccuacgaccccgacaacaaggaagaaagaagcaucgcuaucuacuugggcaucggucugugccugcuuuucaucguccggacccucuuguugcauccugcuauuuucggccugcaucacauuggcaugcagaugagaauugccauguuuucccugaucuacaagaaaacucugaagcucucgagccgcgugcuugacaagauuuccaucggccagcucgugucccugcucuccaacaaucugaacaaguucgacgagggccucgcccuggcccacuucguguggaucgccccucugcaaguggcgcuucugaugggccugaucugggagcugcugcaagccucggcauucugugggcuuggauuccugaucgugcuggcacuguuccaggccggacuggggcggaugaugaugaaguacagggaccagagagccggaaagauuuccgaacggcuggugaucacuucggaaaugaucgaaaacauccagucagugaaggccuacugcugggaagaggccauggaaaagaugauugaaaaccuccggcaaaccgagcugaagcugacccgcaaggccgcuuacgugcgcuauuucaacucguccgcuuucuucuucuccggguucuucgugguguuucucuccgugcuccccuacgcccugauuaagggaaucauccucaggaagaucuucaccaccauuuccuucuguaucgugcuccgcauggccgugacccggcaguucccaugggccgugcagacuugguacgacucccugggagccauuaacaagauccaggacuuccuucaaaagcaggaguacaagacccucgaguacaaccugacuacuaccgaggucgugauggaaaacgucaccgccuuuugggaggagggauuuggcgaacuguucgagaaggccaagcagaacaacaacaaccgcaagaccucgaacggugacgacucccucuucuuuucaaacuucagccugcucgggacgcccgugcugaaggacauuaacuucaagaucgaaagaggacagcuccuggcgguggccggaucgaccggagccggaaagacuucccugcugauggugaucaugggagagcuugaaccuagcgagggaaagaucaagcacuccggccgcaucagcuucuguagccaguuuuccuggaucaugcccggaaccauuaaggaaaacaucaucuucggcguguccuacgaugaauaccgcuaccgguccgugaucaaagccugccagcuggaagaggauauuucaaaguucgcggagaaagauaacaucgugcugggcgaaggggguauuaccuugucggggggccagcgggcuagaaucucgcuggccagagccguguauaaggacgccgaccuguaucuccuggacucccccuucggauaccuggacguccugaccgaaaaggagaucuucgaaucgugcgugugcaagcugauggcuaacaagacucgcauccucgugaccuccaaaauggagcaccugaagaaggcagacaagauucugauucugcaugagggguccuccuacuuuuacggcaccuucucggaguugcagaacuugcagcccgacuucucaucgaagcugauggguugcgacagcuucgaccaguucuccgccgaaagaaggaacucgauccugacggaaaccuugcaccgcuucucuuuggaaggcgacgccccugugucauggaccgagacuaagaagcagagcuucaagcagaccggggaauucggcgaaaagaggaagaacagcaucuugaaccccauuaacuccauccgcaaguucucaaucgugcaaaagacgccacugcagaugaacggcauugaggaggacuccgacgaaccccuugagaggcgccugucccuggugccggacagcgagcagggagaagccauccugccucggauuuccgugaucuccacugguccgacgcuccaagcccggcggcggcaguccgugcugaaccugaugacccacagcgugaaccagggccaaaacauucaccgcaagacuaccgcauccacccggaaagugucccuggcaccucaagcgaaucuuaccgagcucgacaucuacucccggagacugucgcaggaaaccgggcucgaaauuuccgaagaaaucaacgaggaggaucugaaagagugcuucuucgacgauauggagucgauacccgccgugacgacuuggaacacuuaucugcgguacaucacugugcacaagucauugaucuucgugcugauuuggugccuggugauuuuccuggccgaggucgcggccucacugguggugcucuggcuguugggaaacacgccucugcaagacaagggaaacuccacgcacucgagaaacaacagcuaugccgugauuaucacuuccaccuccucuuauuacguguucuacaucuacgucggaguggcggauacccugcucgcgauggguuucuucagaggacugccgcugguccacaccuugaucaccgucagcaagauucuucaccacaagauguugcauagcgugcugcaggcccccauguccacccucaacacucugaaggccggaggcauucugaacagauucuccaaggacaucgcuauccuggacgaucuccugccgcuuaccaucuuugacuucauccagcugcugcugaucgugauuggagcaaucgcagugguggcggugcugcagccuuacauuuucguggccacugugccggucauuguggcguucaucaugcugcgggccuacuuccuccaaaccagccagcagcugaagcaacuggaauccgagggacgaucccccaucuucacucaccuugugacgucguugaagggacuguggacccuccgggcuuucggacggcagcccuacuucgaaacccucuuccacaaggcccugaaccuccacaccgccaauugguuccuguaccuguccacccugcggugguuccagaugcgcaucgagaugauuuucgucaucuucuucaucgcggucacauucaucagcauccugacuaccggagagggagagggacgggucggaauaauccugacccucgccaugaacauuaugagcacccugcagugggcagugaacagcucgaucgacguggacagccugaugcgaagcgucagccgcguguucaaguucaucgacaugccuacugagggaaaacccacuaaguccacuaagcccuacaaaaauggccagcugagcaaggucaugaucaucgaaaacucccacgugaagaaggacgauauuuggcccuccggaggucaaaugaccgugaaggaccugaccgcaaaguacaccgagggaggaaacgccauucucgaaaacaucagcuucuccauuucgccgggacagcgggucggccuucucgggcggaccgguuccgggaagucaacucugcugucggcuuuccuccggcugcugaauaccgagggggaaauccaaauugacggcgugucuugggauuccauuacucugcagcaguggcggaaggccuucggcgugaucccccagaagguguucaucuucucggguaccuuccggaagaaccuggauccuuacgagcaguggagcgaccaagaaaucuggaaggucgccgacgaggucggccugcgcuccgugauugaacaauuuccuggaaagcuggacuucgugcucgucgacgggggauguguccugucgcacggacauaagcagcucaugugccucgcacgguccgugcucuccaaggccaagauucugcugcuggacgaaccuucggcccaccuggauccggucaccuaccagaucaucaggaggacccugaagcaggccuuugccgauugcaccgugauucucugcgagcaccgcaucgaggccaugcuggagugccagcaguuccuggucaucgaggagaacaagguccgccaauacgacuccauucaaaagcuccucaacgagcggucgcuguucagacaagcuauuucaccguccgauagagugaagcucuucccgcaucggaacagcucaaagugcaaaucgaagccgcagaucgcagccuugaaggaagagacugaggaagaggugcaggacacccggcuuuaacggguggcaucccugugaccccuccccagugccucuccuggcccuggaaguugccacuccagugcccaccagccuuguccuaauaaaauuaaguugcaucaagcu

SEQ ID NO: 7 - RNA, 4688 nt, Artificial Sequence
  Synthetic polynucleotide
ggacagaucgccuggagacgccauccacgcuguuuugaccuccauagaagacaccgggaccgauccagccuccgcggccgggaacggugcauuggaacgcggauuccccgugccaagagugacucaccguccuugacacgaugcaacgcucuccucuugaaaaggccucggugguguccaagcucuucuucucguggacuagacccauccugagaaagggguacagacagcgcuuggagcuguccgauaucuaucaaaucccuuccguggacuccgcggacaaccuguccgagaagcucgagagagaaugggacagagaacucgccucaaagaagaacccgaagcugauuaaugcgcuuaggcggugcuuuuucuggcgguucauguucuacggcaucuuccucuaccugggagaggucaccaaggccgugcagccccuguugcugggacggauuauugccuccuacgaccccgacaacaaggaagaaagaagcaucgcuaucuacuugggcaucggucugugccugcuuuucaucguccggacccucuuguugcauccugcuauuuucggccugcaucacauuggcaugcagaugagaauugccauguuuucccugaucuacaagaaaacucugaagcucucgagccgcgugcuugacaagauuuccaucggccagcucgugucccugcucuccaacaaucugaacaaguucgacgagggccucgcccuggcccacuucguguggaucgccccucugcaaguggcgcuucugaugggccugaucugggagcugcugcaagccucggcauucugugggcuuggauuccugaucgugcuggcacuguuccaggccggacuggggcggaugaugaugaaguacagggaccagagagccggaaagauuuccgaacggcuggugaucacuucggaaaugaucgaaaacauccagucagugaaggccuacugcugggaagaggccauggaaaagaugauugaaaaccuccggcaaaccgagcugaagcugacccgcaaggccgcuuacgugcgcuauuucaacucguccgcuuucuucuucuccggguucuucgugguguuucucuccgugcuccccuacgcccugauuaagggaaucauccucaggaagaucuucaccaccauuuccuucuguaucgugcuccgcauggccgugacccggcaguucccaugggccgugcagacuugguacgacucccugggagccauuaacaagauccaggacuuccuucaaaagcaggaguacaagacccucgaguacaaccugacuacuaccgaggucgugauggaaaacgucaccgccuuuugggaggagggauuuggcgaacuguucgagaaggccaagcagaacaacaacaaccgcaagaccucgaacggugacgacucccucuucuuuucaaacuucagccugcucgggacgcccgugcugaaggacauuaacuucaagaucgaaagaggacagcuccuggcgguggccggaucgaccggagccggaaagacuucccugcugauggugaucaugggagagcuugaaccuagcgagggaaagaucaagcacuccggccgcaucagcuucuguagccaguuuuccuggaucaugcccggaaccauuaaggaaaacaucaucuucggcguguccuacgaugaauaccgcuaccgguccgugaucaaagccugccagcuggaagaggauauuucaaaguucgcggagaaagauaacaucgugcugggcgaaggggguauuaccuugucggggggccagcgggcuagaaucucgcuggccagagccguguauaaggacgccgaccuguaucuccuggacucccccuucggauaccuggacguccugaccgaaaaggagaucuucgaaucgugcgugugcaagcugauggcuaacaagacucgcauccucgugaccuccaaaauggagcaccugaagaaggcagacaagauucugauucugcaugagggguccuccuacuuuuacggcaccuucucggaguugcagaacuugcagcccgacuucucaucgaagcugauggguugcgacagcuucgaccaguucuccgccgaaagaaggaacucgauccugacggaaaccuugcaccgcuucucuuuggaaggcgacgccccugugucauggaccgagacuaagaagcagagcuucaagcagaccggggaauucggcgaaaagaggaagaacagcaucuugaaccccauuaacuccauccgcaaguucucaaucgugcaaaagacgccacugcagaugaacggcauugaggaggacuccgacgaaccccuugagaggcgccugucccuggugccggacagcgagcagggagaagccauccugccucggauuuccgugaucuccacugguccgacgcuccaagcccggcggcggcaguccgugcugaaccugaugacccacagcgugaaccagggccaaaacauucaccgcaagacuaccgcauccacccggaaagugucccuggcaccucaagcgaaucuuaccgagcucgacaucuacucccggagacugucgcaggaaaccgggcucgaaauuuccgaagaaaucaacgaggaggaucugaaagagugcuucuucgacgauauggagucgauacccgccgugacgacuuggaacacuuaucugcgguacaucacugugcacaagucauugaucuucgugcugauuuggugccuggugauuuuccuggccgaggucgcggccucacugguggugcucuggcuguugggaaacacgccucugcaagacaagggaaacuccacgcacucgagaaacaacagcuaugccgugauuaucacuuccaccuccucuuauuacguguucuacaucuacgucggaguggcggauacccugcucgcgauggguuucuucagaggacugccgcugguccacaccuugaucaccgucagcaagauucuucaccacaagauguugcauagcgugcugcaggcccccauguccacccucaacacucugaaggccggaggcauucugaacagauucuccaaggacaucgcuauccuggacgaucuccugccgcuuaccaucuuugacuucauccagcugcugcugaucgugauuggagcaaucgcagugguggcggugcugcagccuuacauuuucguggccacugugccggucauuguggcguucaucaugcugcgggccuacuuccuccaaaccagccagcagcugaagcaacuggaauccgagggacgaucccccaucuucacucaccuugugacgucguugaagggacuguggacccuccgggcuuucggacggcagcccuacuucgaaacccucuuccacaaggcccugaaccuccacaccgccaauugguuccuguaccuguccacccugcggugguuccagaugcgcaucgagaugauuuucgucaucuucuucaucgcggucacauucaucagcauccugacuaccggagagggagagggacgggucggaauaauccugacccucgccaugaacauuaugagcacccugcagugggcagugaacagcucgaucgacguggacagccugaugcgaagcgucagccgcguguucaaguucaucgacaugccuacugagggaaaacccacuaaguccacuaagcccuacaaaaauggccagcugagcaaggucaugaucaucgaaaacucccacgugaagaaggacgauauuuggcccuccggaggucaaaugaccgugaaggaccugaccgcaaaguacaccgagggaggaaacgccauucucgaaaacaucagcuucuccauuucgccgggacagcgggucggccuucucgggcggaccgguuccgggaagucaacucugcugucggcuuuccuccggcugcugaauaccgagggggaaauccaaauugacggcgugucuugggauuccauuacucugcagcaguggcggaaggccuucggcgugaucccccagaagguguucaucuucucggguaccuuccggaagaaccuggauccuuacgagcaguggagcgaccaagaaaucuggaaggucgccgacgaggucggccugcgcuccgugauugaacaauuuccuggaaagcuggacuucgugcucgucgacgggggauguguccugucgcacggacauaagcagcucaugugccucgcacgguccgugcucuccaaggccaagauucugcugcuggacgaaccuucggcccaccuggauccggucaccuaccagaucaucaggaggacccugaagcaggccuuugccgauugcaccgugauucucugcgagcaccgcaucgaggccaugcuggagugccagcaguuccuggucaucgaggagaacaagguccgccaauacgacuccauucaaaagcuccucaacgagcggucgcuguucagacaagcuauuucaccguccgauagagugaagcucuucccgcaucggaacagcucaaagugcaaaucgaagccgcagaucgcagccuugaaggaagagacugaggaagaggugcaggacacccggcuuuaaggguggcaucccugugaccccuccccagugccucuccuggcccuggaaguugccacuccagugcccaccagccuuguccuaauaaaauuaaguugcaucaaagcu

SEQ ID NO: 8 - DNA, 4443 bp, Artificial Sequence
  Synthetic polynucleotide
atgcagaggagcccactggagaaagcctccgtggtgagtaaactcttttttagttggaccagacccatcctgcgaaaaggatacaggcagcgcctcgagttgtcagatatctaccagattccttctgtggactcagctgacaatttgagtgagaagctggagcgggagtgggatagagagctggcgagcaaaaaaaaccccaagcttatcaatgctctgcgccgctgctttttctggaggttcatgttttatgggatcttcctgtacctgggggaggtcaccaaagctgttcagccgctccttcttggccgcatcatcgccagctatgaccctgataataaagaagaaaggtctattgctatttatctgggaattggcctctgcttgctcttcatcgtccgcacccttctgctgcaccctgccatttttggccttcaccacatcggcatgcaaatgagaattgccatgttctccctcatttacaaaaagaccctgaaactttcctcaagagtgttagataaaatatccattggtcagctggtcagcctgctgtccaacaatcttaacaaatttgatgaaggcttggcgctggcccacttcgtgtggattgcacctctgcaggtggccctgttgatgggacttatatgggagctgcttcaagcctctgctttctgtgggctgggctttttgattgtactggcactttttcaggctgggctcggaagaatgatgatgaaatacagagatcagcgggccgggaagatatcagagcgacttgtgatcaccagtgaaatgattgaaaatattcagagcgtgaaagcctactgctgggaagaagccatggagaagatgattgagaacctgaggcagacagagctcaagctcactcggaaggctgcttatgttcgctatttcaacagcagcgccttcttcttcagtggcttctttgttgtcttcctgtctgttctgccatatgcactgataaaaggcattattttacgaaagatcttcaccaccatcagtttttgcatcgttctcaggatggccgtcacaagacagttcccctgggctgtgcagacctggtacgattccttgggggccatcaacaagattcaagatttcttgcaaaaacaagaatataaaactttagaatacaacctcaccaccactgaagtggtcatggaaaatgtgacagccttttgggaggagggttttggagaattgttcgagaaggcaaagcagaataacaacaacaggaagacgagcaatggggacgactctctcttcttcagcaacttttcactgctcgggacccctgtgttgaaagatataaacttcaagatcgagaggggccagctcttggctgtggcaggctccactggagctggtaaaacatctcttctcatggtgatcatgggggaactggagccttccgaaggaaaaatcaagcacagtgggagaatctcattctgcagccagttttcctggatcatgcccggcaccattaaggaaaacatcatatttggagtgtcctatgatgagtaccgctaccggtcagtcatcaaagcctgtcagttggaggaggacatctccaagtttgcagagaaagacaacattgtgcttggagaggggggtatcactctttctggaggacaaagagccaggatctctttggcccgggcagtctacaaggatgcagacctctacttgttggacagtcccttcggctacctcgacgtgctgactgaaaaagaaatttttgaaagctgtgtgtgcaaactgatggcaaacaagaccaggattcttgtcaccagcaagatggaacatctgaagaaagcggacaaaattctgattctgcatgaagggagctcctacttctatggaacatttagcgagcttcagaacctacagccagacttctcctccaaattaatgggctgtgactccttcgaccagttctctgcagaaagaagaaactctatactcacagagaccctccaccgcttctcccttgagggagatgccccagtttcttggacagaaaccaagaagcagtcctttaagcagactggcgagtttggtgaaaagaggaaaaattcaattctcaatccaattaacagtattcgcaagttcagcattgtccagaagacacccctccagatgaatggcatcgaagaagatagtgacgagccgctggagagacggctgagtctggtgccagattcagaacagggggaggccatcctgccccggatcagcgtcatttccacaggccccacattacaagcacggcgccggcagagtgttttaaatctcatgacccattcagtgaaccagggccaaaatatccacaggaagactacagcttctacccggaaagtgtctctggcccctcaggccaatctgaccgagctggacatctacagcaggaggctctcccaggaaacagggctggaaatatctgaagagattaatgaagaggatcttaaagagtgcttctttgatgacatggagagcatccccgcggtgaccacatggaacacctaccttagatatattactgtccacaagagcctcatatttgtcctcatctggtgcctggttattttcctcgctgaggtggcggccagtcttgttgtgctctggctgctgggcaacactcctctccaggacaagggcaatagtactcacagcagaaataattcttatgccgtcatcattacaagcacctccagctactacgtgttctacatctatgtgggcgtggctgacaccctcctggccatgggtttcttccggggcctgcctttggtgcacaccctcatcacagtgtcaaaaattctgcaccataaaatgcttcattctgtcctgcaggcacccatgagcactttgaacacattgaaggctggcggcatcctcaacagattttctaaagatattgctatcctggatgatctcctccccctgacaatctttgactttatccagcttctgctgatcgtgattggagccatagcagtggttgctgtcctgcagccctacatttttgtggccaccgtgcccgtgattgttgcctttattatgctcagagcttacttcctgcaaacttctcaacagctcaaacagctagaatctgagggccggagccccatttttacccacctggtgacttccctgaagggactgtggactctgagagcattcgggcgacagccttactttgagacactgttccacaaggccctgaacttgcacactgccaactggtttctttacctgagcacactccgctggttccagatgcggatagagatgatcttcgtcatcttttttatagctgtaaccttcatttctatccttacaacaggagaaggagagggcagggtgggaatcatcctcacgctggctatgaacataatgtccaccttgcagtgggccgtgaattccagtatagatgtggattctctaatgaggagtgtctcccgggtgtttaaattcattgatatgcctactgaggggaaacccaccaagtcaacaaaaccttataagaatggacagctgagcaaggtgatgataattgagaacagccacgtgaagaaggatgacatttggcccagcgggggccagatgactgtgaaggacctgacggccaagtacaccgaaggtggaaatgccattttggaaaacatcagcttctcaatctctcctgggcagagagttggattgctgggtcgcacgggcagcggcaaatcaaccctgctcagtgccttccttcggctcctgaatacagaaggcgaaatccaaattgacggggtgagctgggacagcatcaccctgcagcagtggagaaaagcatttggggtcattccacagaaagttttcatcttctctggcactttcagaaagaacctggacccctatgagcagtggagcgaccaggagatctggaaggttgcagatgaagttggcctgcggagtgtgatagaacaatttcctggcaagctggattttgtgctggtagatggaggctgcgtgctgtcccacggccacaaacagctgatgtgcctcgcccgctccgttctttcaaaggccaaaatcttgcttttggatgagcccagtgctcacctcgacccagtgacctatcagataatccgcaggaccttaaagcaagcttttgccgactgcaccgtcatactgtgtgagcaccggattgaagcaatgctggaatgccagcagtttctggtgatcgaggagaataaggtccggcagtacgacagcatccagaagttgttgaatgagcgcagccttttccgccaggccatctccccatctgacagagtcaagctgtttccacataggaactcctctaagtgcaagtccaagccccagatcgctgccctcaaggaggaaactgaggaagaggtgcaggatacccgcctgtga

SEQ ID NO: 9 - DNA, 4443 bp, Artificial Sequence
  Synthetic polynucleotide
atgcagaggagcccactggagaaagcctccgtggtgagtaaactcttttttagttggaccagacccatcctgcgaaaaggatacaggcagcgcctcgagttgtctgatatctaccagattccttctgtggactcagctgacaatttgagtgagaagctggagcgggagtgggatagagagctggcgagcaaaaaaaaccccaagcttatcaatgctctgcgccgctgctttttctggaggttcatgttttatgggatcttcctgtacctgggggaggtcaccaaagctgttcagccgctccttcttggccgcatcatcgccagctatgaccctgataataaagaagaaaggtctattgctatttatctgggaattggcctctgcttgctcttcatcgtccgcacccttctgctgcaccctgccatttttggccttcaccacatcggcatgcaaatgagaattgccatgttctccctcatttacaaaaagaccctgaaactttcctcaagagtgttagataaaatatccattggtcagctggtcagcctgctgtccaacaatcttaacaaatttgatgaaggcttggcgctggcccacttcgtgtggattgcacctctgcaggtggccctgttgatgggacttatatgggagctgcttcaagcctctgctttctgtgggctgggctttttgattgtactggcactttttcaggctgggctcggaagaatgatgatgaaatacagagatcagcgggccgggaagatttcagagcgacttgtgatcaccagtgaaatgattgaaaatattcagagcgtgaaagcctactgctgggaagaagccatggagaagatgattgagaacctgaggcagacagagctcaagctcactcggaaggctgcttatgttcgctatttcaacagcagcgccttcttcttcagtggcttctttgttgtcttcctgtctgttctgccatatgcactgataaaaggcattattttacgaaagatcttcaccaccatcagtttttgcatcgttctcaggatggccgtcacaagacagttcccctgggctgtgcagacctggtacgattccttgggggccatcaacaagattcaagatttcttgcaaaaacaagaatataaaactttagaatacaacctcaccaccactgaagtggtcatggaaaatgtgacagccttttgggaggagggttttggagaattgttcgagaaggcaaagcagaataacaacaacaggaagacgagcaatggggacgactctctcttcttcagcaacttttcactgctcgggacccctgtgttgaaagatataaacttcaagatcgagaggggccagctcttggctgtggcaggctccactggagctggtaaaacatctcttctcatggtgatcatgggggaactggagccttccgaaggaaaaatcaagcacagtgggagaatctcattctgcagccagttttcctggatcatgcccggcaccattaaggaaaacatcatatttggagtgtcctatgatgagtaccgctaccggtcagtcatcaaagcctgtcagttggaggaggacatctccaagtttgcagagaaagacaacattgtgcttggagaggggggtatcactctttctggaggacaaagagccaggatctctttggcccgggcagtctacaaggatgcagacctctacttgttggacagtcccttcggctacctcgacgtgctgactgaaaaagaaatttttgaaagctgtgtgtgcaaactgatggcaaacaagaccaggattcttgtcaccagcaagatggaacatctgaagaaagcggacaaaattctgattctgcatgaagggagctcctacttctatggaacatttagcgagcttcagaacctacagccagacttctcctccaaattaatgggctgtgactccttcgaccagttctctgcagaaagaagaaactctatactcacagagaccctccaccgcttctcccttgagggagatgccccagtttcttggacagaaaccaagaagcagtcctttaagcagactggcgagtttggtgaaaagaggaaaaattcaattctcaatccaattaacagtattcgcaagttcagcattgtccagaagacacccctccagatgaatggcatcgaagaagatagtgacgagccgctggagagacggctgagtctggtgccagattcagaacagggggaggccatcctgccccggatcagcgtcatttccacaggccccacattacaagcacggcgccggcagagtgttttaaatctcatgacccattcagtgaaccagggccaaaatatccacaggaagactacagcttctacccggaaagtgtctctggcccctcaggccaatctgaccgagctggacatctacagcaggaggctctcccaggaaacagggctggaaatatctgaagagattaatgaagaggatcttaaagagtgcttctttgatgacatggagagcatccccgcggtgaccacatggaacacctaccttagatatattactgtccacaagagcctcatatttgtcctcatctggtgcctggttattttcctcgctgaggtggcggccagtcttgttgtgctctggctgctgggcaacactcctctccaggacaagggcaatagtactcacagcagaaataattcttatgccgtcatcattacaagcacctccagctactacgtgttctacatctatgtgggcgtggctgacaccctcctggccatgggtttcttccggggcctgcctttggtgcacaccctcatcacagtgtcaaaaattctgcaccataaaatgcttcattctgtcctgcaggcacccatgagcactttgaacacattgaaggctggcggcatcctcaacagattttctaaagatattgctatcctggatgatctcctccccctgacaatctttgactttatccagcttctgctgatcgtgattggagccatagcagtggttgctgtcctgcagccctacatttttgtggccaccgtgcccgtgattgttgcctttattatgctcagagcttacttcctgcaaacttctcaacagctcaaacagctagaatctgagggccggagccccatttttacccacctggtgacttccctgaagggactgtggactctgagagcattcgggcgacagccttactttgagacactgttccacaaggccctgaacttgcacactgccaactggtttctttacctgagcacactccgctggttccagatgcggatagagatgatcttcgtcatcttttttatagctgtaaccttcatttctatccttacaacaggagaaggagagggcagggtgggaatcatcctcacgctggctatgaacataatgtccaccttgcagtgggccgtgaattccagtatagatgtggattctctaatgaggagtgtctcccgggtgtttaaattcattgatatgcctactgaggggaaacccaccaagtcaacaaaaccttataagaatggacagctgagcaaggtgatgataattgagaacagccacgtgaagaaggatgacatttggcccagcgggggccagatgactgtgaaggacctgacggccaagtacaccgaaggtggaaatgccattttggaaaacatcagcttctcaatctctcctgggcagagagttggattgctgggtcgcacgggcagcggcaaatcaaccctgctcagtgccttccttcggctcctgaatacagaaggcgaaatccaaattgacggggtgagctgggacagcatcaccctgcagcagtggagaaaagcatttggggtcattccacagaaagttttcatcttctctggcactttcagaaagaacctggacccctatgagcagtggagcgaccaggagatctggaaggttgcagatgaagttggcctgcggagtgtgatagaacaatttcctggcaagctggattttgtgctggtagatggaggctgcgtgctgtcccacggccacaaacagctgatgtgcctcgcccgctccgttctttcaaaggccaaaatcttgcttttggatgagcccagtgctcaccttgacccagtgacctatcagataatccgcaggaccttaaagcaagcttttgccgactgcaccgtcatactgtgtgagcaccggattgaagcaatgctggaatgccagcagtttctggtgatcgaggagaataaggtccggcagtacgacagcatccagaagttgttgaatgagcgcagccttttccgccaggccatctccccatctgacagagtcaagctgtttccacataggaactcctctaagtgcaagtccaagccccagatcgctgccctcaaggaggaaactgaggaagaggtgcaggatacccgcctgtga

SEQ ID NO: 10 - DNA, 4443 bp, Artificial Sequence
  Synthetic polynucleotide
atgcagaggagcccactggagaaagcctccgtggtgagtaaactcttttttagttggaccagacccatcctgcgaaaaggatacaggcagcgcctcgagttgtcagatatctaccagattccttctgtggactcagctgacaatttgagtgagaagctggagcgggagtgggatagagagctggcgagcaaaaaaaaccccaagcttatcaatgctctgcgccgctgctttttctggaggttcatgttttatgggatcttcctgtacctgggggaggtcaccaaagctgttcagccgctccttcttggccgcatcatcgccagctatgaccctgataataaagaagaaaggtctattgctatttatctgggaattggcctctgcttgctcttcatcgtccgcacccttctgctgcaccctgccatttttggccttcaccacatcggcatgcaaatgagaattgccatgttctccctcatttacaaaaagaccctgaaactttcctcaagagtgttagataaaatatccattggtcagctggtcagcctgctgtccaacaatcttaacaaatttgatgaaggcttggcgctggcccacttcgtgtggattgcacctctgcaggtggccctgttgatgggacttatatgggagctgcttcaagcctctgctttctgtgggctgggctttttgattgtactggcactttttcaggctgggctcggaagaatgatgatgaaatacagagatcagcgggccgggaagatatcagagcgacttgtgatcaccagtgaaatgattgaaaatattcagagcgtgaaagcctactgctgggaagaagccatggagaagatgattgagaacctgaggcagacagagctcaagctcactcggaaggctgcttatgttcgctatttcaacagcagcgccttcttcttcagtggcttctttgttgtcttcctgtctgttctgccatatgcactgataaaaggcattattttacgaaagatcttcaccaccatcagtttttgcatcgttctcaggatggccgtcacaagacagttcccctgggctgtgcagacctggtacgattccttgggggccatcaacaagattcaagatttcttgcaaaaacaagaatataaaactttagaatacaacctcaccaccactgaagtggtcatggaaaatgtgacagccttttgggaggagggttttggagaattgttcgagaaggcaaagcagaataacaacaacaggaagacgagcaatggggacgactctctcttcttcagcaacttttcactgctcgggacccctgtgttgaaagatataaacttcaagatcgagaggggccagctcttggctgtggcaggctccactggagctggtaaaacatctcttctcatggtgatcatgggggaactggagccttccgaaggaaaaatcaagcacagtgggagaatctcattctgcagccagttttcctggatcatgcccggcaccattaaggaaaacatcatatttggagtgtcctatgatgagtaccgctaccggtcagtcatcaaagcctgtcagttggaggaggacatctccaagtttgcagagaaagacaacattgtgcttggagaggggggtatcactctttctggaggacaaagagccaggatctctttggcccgggcagtctacaaggatgcagacctctacttgttggacagtcccttcggctacctcgacgtgctgactgaaaaagaaatttttgaaagctgtgtgtgcaaactgatggcaaacaagaccaggattcttgtcaccagcaagatggaacatctgaagaaagcggacaaaattctgattctgcatgaagggagctcctacttctatggaacatttagcgagcttcagaacctacagccagacttctcctccaaattaatgggctgtgactccttcgaccagttctctgcagaaagaagaaactctatactcacagagaccctccaccgcttctcccttgagggagatgccccagtttcttggacagaaaccaagaagcagtcctttaagcagactggcgagtttggtgaaaagaggaaaaattcaattctcaatccaattaacagtattcgcaagttcagcattgtccagaagacacccctccagatgaatggcatcgaagaagatagtgacgagccgctggagagacggctgagtctggtgccagattcagaacagggggaggccatcctgccccggatcagcgtcatttccacaggccccacattacaagcacggcgccggcagagtgttttaaatctcatgacccattcagtgaaccagggccaaaatatccacaggaagactacagcttctacccggaaagtgtctctggcccctcaggccaatctgaccgagctggacatctacagcaggaggctctcccaggaaacagggcttgaaatatctgaagagattaatgaagaggatcttaaagagtgcttctttgatgacatggagagcatccccgcggtgaccacatggaacacctaccttagatatattactgtccacaagagcctcatatttgtcctcatctggtgcctggttattttcctcgctgaggtggcggccagtcttgttgtgctctggctgctgggcaacactcctctccaggacaagggcaatagtacacacagcagaaataattcttatgccgtcatcattacaagcacctccagctactacgtgttctacatctatgtgggcgtggctgacaccctcctggccatgggtttcttccggggcctgcctttggtgcacaccctcatcacagtgtcaaaaattctgcaccataaaatgcttcattctgtcctgcaggcacccatgagcactttgaacacattgaaggctggcggcatcctcaacagattttctaaagatattgctatcctggatgatctcctccccctgacaatctttgactttatccagcttctgctgatcgtgattggagccatagcagtggttgctgtcctgcagccctacatttttgtggccaccgtgcccgtgattgttgcctttattatgctcagagcttacttcctgcaaacttctcaacagctcaaacagctagaatctgagggccggagccccatttttacccacctggtgacttccctgaagggactgtggactctgagagcattcgggcgacagccttactttgagacactgttccacaaggccctgaacttgcacactgccaactggtttctttacctgagcacactccgctggttccagatgcggatagagatgatcttcgtcatcttttttatagctgtaaccttcatttctatccttacaacaggagaaggagagggcagggtgggaatcatcctcacgctggctatgaacataatgtccaccttgcagtgggccgtgaattccagtatagatgtggattctctaatgaggagtgtctcccgggtgtttaaattcattgatatgcctactgaggggaaacccaccaagtcaacaaaaccttataagaatggacagctgagcaaggtgatgataattgagaacagccacgtgaagaaggatgacatttggcccagcgggggccagatgactgtgaaggacctgacggccaagtacaccgaaggtggaaatgccattttggaaaacatcagcttctcaatctctcctgggcagagagttggattgctgggtcgcacgggcagcggcaaatcaaccctgctcagtgccttccttcggctcctgaatacagaaggcgaaatccaaattgacggggtgagctgggacagcatcaccctgcagcagtggagaaaagcatttggggtcattccacagaaagttttcatcttctctggcactttcagaaagaacctggacccctatgagcagtggagcgaccaggagatctggaaggttgcagatgaagttggcctgcggagtgtgatagaacaatttcctggcaagctggattttgtgctggtagatggaggctgcgtgctgtcccacggccacaaacagctgatgtgcctcgcccgctccgttctttcaaaggccaaaatcttgcttttggatgagcccagtgctcaccttgacccagtgacctatcagataatccgcaggaccttaaagcaagcttttgccgactgcaccgtcatactgtgtgagcaccggattgaagcaatgctggaatgccagcagtttctggtgatcgaggagaataaggtccggcagtacgacagcatccagaagttgttgaatgagcgcagccttttccgccaggccatctccccatctgacagagtcaagctgtttccacataggaactcctctaagtgcaagtccaagccccagatcgctgccctcaaggaggaaactgaggaagaggtgcaggatacccgcctgtga

SEQ ID NO: 11 - DNA, 4443 bp, Artificial Sequence
  Synthetic polynucleotide
atgcagaggagcccactggagaaagcctccgtggtgagtaaactcttttttagttggaccagacccatcctgcgaaaaggatacaggcagcgcctcgagttgtcagatatctaccagattccttctgtggactcagctgacaatttgagtgagaagctggagcgggagtgggatagagagctggcgagcaaaaaaaaccccaagcttatcaatgctctgcgccgctgctttttctggaggttcatgttttatgggatcttcctgtacctgggggaggtcaccaaagctgttcagccgctccttcttggccgcatcatcgccagctatgaccctgataataaagaagaaaggtctattgctatttatctgggaattggcctctgcttgctcttcatcgtccgcacccttctgctgcaccctgccatttttggccttcaccacatcggcatgcaaatgagaattgccatgttctccctcatttacaaaaagaccctgaaactttcctcaagagtgttagataaaatatccattggtcagctggtcagcctgctgtccaacaatcttaacaaatttgatgaaggcttggcgctggcccacttcgtgtggattgcacctctgcaggtggccctgttgatgggacttatatgggagctgcttcaagcctctgctttctgtgggctgggctttttgattgtactggcactttttcaggctgggctcggaagaatgatgatgaaatacagagatcagcgggccgggaagatatcagagcgacttgtgatcaccagtgaaatgattgaaaatattcagagcgtgaaagcctactgctgggaagaagccatggagaagatgattgagaacctgaggcagacagagctcaagctcactcggaaggctgcttatgttcgctatttcaacagcagcgccttcttcttcagtggcttctttgttgtcttcctgtctgttctgccatatgcactgataaaaggcattattttacgaaagatcttcaccaccatcagtttttgcatcgttctcaggatggccgtcacaagacagttcccctgggctgtgcagacctggtacgattccttgggggccatcaacaagattcaagatttcttgcaaaaacaagaatataaaactttagaatacaacctcaccaccactgaagtggtcatggaaaatgtgacagccttttgggaggagggttttggagaattgttcgagaaggcaaagcagaataacaacaacaggaagacgagcaatggggacgactctctcttcttcagcaacttttcactgctcgggacccctgtgttgaaagatataaacttcaagatcgagaggggccagctcttggctgtggcaggctccactggagctggtaaaacatctcttctcatggtgatcatgggggaactggagccttccgaaggaaaaatcaagcacagtgggagaatctcattctgcagccagttttcctggatcatgcccggcaccattaaggaaaacatcatatttggagtgtcctatgatgagtaccgctaccggtcagtcatcaaagcctgtcagttggaggaggacatctccaagtttgcagagaaagacaacattgtgcttggagaggggggtatcactctttctggaggacaaagagccaggatctctttggcccgggcagtctacaaggatgcagacctctacttgttggacagtcccttcggctacctcgacgtgctgactgaaaaagaaatttttgaaagctgtgtgtgcaaactgatggcaaacaagaccaggattcttgtcaccagcaagatggaacatctgaagaaagcggacaaaattctgattctgcatgaagggagctcctacttctatggaacatttagcgagcttcagaacctacagccagacttctcctccaaattaatgggctgtgactccttcgaccagttctctgcagaaagaagaaactctatactcacagagaccctccaccgcttctcccttgagggagatgccccagtttcttggacagaaaccaagaagcagtcctttaagcagactggcgagtttggtgaaaagaggaaaaattcaattctcaatccaattaacagtattcgcaagttcagcattgtccagaagacacccctccagatgaatggcatcgaagaagatagtgacgagccgctggagagacggctgagtctggtgccagattcagaacagggggaggccatcctgccccggatcagcgtcatttccacaggccccacattacaagcacggcgccggcagagtgttttaaatctcatgacccattcagtgaaccagggccaaaatatccacaggaagactacagcttctacccggaaagtgtctctggcccctcaggccaatctgaccgagctggacatctacagcaggaggctctcccaggaaacagggctggaaatatctgaagagattaatgaagaggatcttaaagagtgcttctttgatgacatggagagcatccccgcggtgaccacatggaacacctaccttagatatattactgtccacaagagcctcatatttgtcctcatctggtgcctggttattttcctcgctgaggtggcggccagtcttgttgtgctctggctgctgggcaacactcctctccaggacaagggcaatagtactcacagcagaaataattcttatgccgtcatcattacaagcacctccagctactacgtgttctacatctatgtgggcgtggctgacaccctcctggccatgggtttcttccggggcctgcctttggtgcacaccctcatcacagtgtcaaaaattctgcaccataaaatgcttcattctgtcctgcaggcacccatgagcactttgaacacattgaaggctggcggcatcctcaacagattttctaaagatattgctatcctggatgatctcctccccctgacaatctttgactttatccagcttctgctgatcgtgattggagccatagcagtggttgctgtcctgcagccctacatttttgtggccaccgtgcccgtgattgttgcctttattatgctcagagcttacttcctgcaaacttctcaacagctcaaacagctagaatctgagggccggagccccatttttacccacctggtgacttccctgaagggactgtggactctgagagcattcgggcgacagccttactttgagacactgttccacaaggccctgaacttgcacactgccaactggtttctttacctgagcacactccgctggttccagatgcggatagagatgatcttcgtcatcttttttatagctgtaaccttcatttctatccttacaacaggagaaggagagggcagggtgggaatcatcctcacgctggctatgaacataatgtccaccttgcagtgggccgtgaattccagtatagatgtggattctctaatgaggagtgtctcccgggtgtttaaattcattgatatgccaactgaggggaaacccaccaagtcaacaaaaccttataagaatggacagctgagcaaggtgatgataattgagaacagccacgtgaagaaggatgacatttggcccagcgggggccagatgactgtgaaggacctgacggccaagtacaccgaaggtggaaatgccattttggaaaacatcagcttctcaatctctcctgggcagagagttggattgctgggtcgcacgggcagcggcaaatcaaccctgctcagtgccttccttcggctcctgaatacagaaggcgaaatccaaattgacggggtgagctgggacagcatcaccctgcagcagtggagaaaagcatttggggtcattccacagaaagttttcatcttctctggcactttcagaaagaacctggacccctatgagcagtggagcgaccaggagatctggaaggttgcagatgaagttggcctgcggagtgtgatagaacaatttcctggcaagctggattttgtgctggtagatggaggctgcgtgctgtcccacggccacaaacagctgatgtgcctcgcccgctccgttctttcaaaggccaaaatcttgcttttggatgagcccagtgctcacctcgacccagtgacctatcagataatccgcaggaccttaaagcaagcttttgccgactgcaccgtcatactgtgtgagcaccggattgaagcaatgctggaatgccagcagtttctggtgatcgaggagaataaggtccggcagtacgacagcatccagaagttgttgaatgagcgcagccttttccgccaggccatctccccatctgacagagtcaagctgtttccacataggaactcctctaagtgcaagtccaagccccagatcgctgccctcaaggaggaaactgaggaagaggtgcaggatacccgcctgtga

SEQ ID NO: 12 - DNA, 4443 bp, Artificial Sequence
  Synthetic polynucleotide
atgcagaggagcccactggagaaagcctccgtggtgagtaaactcttttttagttggaccagacccatcctgcgaaaaggatacaggcagcgcctcgagttgtcagatatctaccagattccttctgtggactcagctgacaatttgagtgagaagctggagcgggagtgggatagagagctggcgagcaaaaaaaaccccaagcttatcaatgctctgcgccgctgctttttctggaggttcatgttttatgggatcttcctgtacctgggggaggtcaccaaagctgttcagccgctccttcttggccgcatcatcgccagctatgaccctgataataaagaagaaaggtctattgctatttatctgggaattggcctctgcttgctcttcatcgtccgcacccttctgctgcaccctgccatttttggccttcaccacatcggcatgcaaatgagaattgccatgttctccctcatttacaaaaagaccctgaaactttcctcaagagtgttagataaaatatccattggtcagctggtcagcctgctgtccaacaatcttaacaaatttgatgaaggcttggcgctggcccacttcgtgtggattgcacctctgcaggtggccctgttgatgggacttatatgggagctgcttcaagcctctgctttctgtgggctgggctttttgattgtactggcactttttcaggctgggctcggaagaatgatgatgaaatacagagatcagcgggccgggaagatatcagagcgacttgtgatcaccagtgaaatgattgaaaatattcagagcgtgaaagcctactgctgggaagaagccatggagaagatgattgagaacctgaggcagacagagctcaagctcactcggaaggctgcttatgttcgctatttcaacagcagcgccttcttcttcagtggcttctttgttgtcttcctgtctgttctgccatatgcactgataaaaggcattattttacgaaagatcttcaccaccatcagtttttgcatcgttctcaggatggccgtcacaagacagttcccctgggctgtgcagacctggtacgattccttgggggccatcaacaagattcaagatttcttgcaaaaacaagaatataaaactttagaatacaacctcaccaccactgaagtggtcatggaaaatgtgacagccttttgggaggagggttttggagaattgttcgagaaggcaaagcagaataacaacaacaggaagacgagcaatggggacgactctctcttcttcagcaacttttcactgctcgggacccctgtgttgaaagatataaacttcaagatcgagaggggccagctcttggctgtggcaggctccactggagctggtaaaacatctcttctcatggtgatcatgggggaactggagccttccgaaggaaaaatcaagcacagtgggagaatctcattctgcagccagttttcctggatcatgcccggcaccattaaggaaaacatcatatttggagtgtcctatgatgagtaccgctaccggtcagtcatcaaagcctgtcagttggaggaggacatctccaagtttgcagagaaagacaacattgtgcttggagaggggggtatcactctttctggaggacaaagagccaggatctctttggcccgggcagtctacaaggatgcagacctctacttgttggacagtcccttcggctacctcgacgtgctgactgaaaaagaaatttttgaaagctgtgtgtgcaaactgatggcaaacaagaccaggattcttgtcaccagcaagatggaacatctgaagaaagcggacaaaattctgattctgcatgaagggagctcctacttctatggaacatttagcgagcttcagaacctacagccagacttctcctccaaattaatgggctgtgactccttcgaccagttctctgcagaaagaagaaactctatactcacagagaccctccaccgcttctcccttgagggagatgccccagtttcttggacagaaaccaagaagcagtcctttaagcagactggcgagtttggtgaaaagaggaaaaattcaattctcaatcctattaacagtattcgcaagttcagcattgtccagaagacacccctccagatgaatggcatcgaagaagatagtgacgagccgctggagagacggctgagtctggtgccagattcagaacagggggaggccatcctgccccggatcagcgtcatttccacaggccccacattacaagcacggcgccggcagagtgttttaaatctcatgacccattcagtgaaccagggccaaaatatccacaggaagactacagcttctacccggaaagtgtctctggcccctcaggccaatctgaccgagctggacatctacagcaggaggctctcccaggaaacagggcttgaaatatctgaagagattaatgaagaggatcttaaagagtgcttctttgatgacatggagagcatccccgcggtgaccacatggaacacctaccttagatatattactgtccacaagagcctcatatttgtcctcatctggtgcctggttattttcctcgctgaggtggcggccagtcttgttgtgctctggctgctgggcaacactcctctccaggacaagggcaatagtactcacagcagaaataattcttatgccgtcatcattacaagcacctccagctactacgtgttctacatctatgtgggcgtggctgacaccctcctggccatgggtttcttccggggcctgcctttggtgcacaccctcatcacagtgtcaaaaattctgcaccataaaatgcttcattctgtcctgcaggcacccatgagcactttgaacacattgaaggctggcggcatcctcaacagattttctaaagatattgctatcctggatgatctcctccccctgacaatctttgactttatccagcttctgctgatcgtgattggagccatagcagtggttgctgtcctgcagccctacatttttgtggccaccgtgcccgtgattgttgcctttattatgctcagagcttacttcctgcaaacttctcaacagctcaaacagctagaatctgagggccggagccccatttttacccacctggtgacttccctgaagggactgtggactctgagagcattcgggcgacagccttactttgagacactgttccacaaggccctgaacttgcacactgccaactggtttctttacctgagcacactccgctggttccagatgcggatagagatgatcttcgtcatcttttttatagctgtaaccttcatttctatccttacaacaggagaaggagagggcagggtgggaatcatcctcacgctggctatgaacataatgtccaccttgcagtgggccgtgaattccagtatagatgtggattctctaatgaggagtgtctcccgggtgtttaaattcattgatatgcctactgaggggaaacccaccaagtcaacaaaaccttataagaatggacagctgagcaaggtgatgataattgagaacagccacgtgaagaaggatgacatttggcccagcgggggccagatgactgtgaaggacctgacggccaagtacaccgaaggtggaaatgccattttggaaaacatcagcttctcaatctctcctgggcagagagttggattgctgggtcgcacgggcagcggcaaatcaaccctgctcagtgccttccttcggctcctgaatacagaaggcgaaatccaaattgacggggtgagctgggacagcatcaccctgcagcagtggagaaaagcatttggggtcattccacagaaagttttcatcttctctggcactttcagaaagaacctggacccctatgagcagtggagcgaccaggagatctggaaggttgcagatgaagttggcctgcggagtgtgatagaacaatttcctggcaagctggattttgtgctggtagatggaggctgcgtgctgtcccacggccacaaacagctgatgtgcctcgcccgctccgttctttcaaaggccaaaatcttgcttttggatgagcccagtgctcacctcgacccagtgacctatcagataatccgcaggaccttaaagcaagcttttgccgactgcaccgtcatactgtgtgagcaccggattgaagcaatgctggaatgccagcagtttctggtgatcgaggagaataaggtccggcagtacgacagcatccagaagttgttgaatgagcgcagccttttccgccaggccatctccccatctgacagagtcaagctgtttccacataggaactcctctaagtgcaagtccaagccccagatcgctgccctcaaggaggaaactgaggaagaggtgcaggatacccgcctgtga

SEQ ID NO: 13 - DNA, 4443 bp, Artificial Sequence
  Synthetic polynucleotide
atgcagaggagcccactggagaaagcctccgtggtgagtaaactcttttttagttggaccagacccatcctgcgaaaaggatacaggcagcgcctcgagttgtcagatatctaccagattccttctgtggactcagctgacaatttgagtgagaagctggagcgggagtgggatagagagctggcgagcaaaaaaaaccccaagcttatcaatgctctgcgccgctgctttttctggaggttcatgttttatgggatcttcctgtacctgggggaggtcaccaaagctgttcagccgctccttcttggccgcatcatcgccagctatgaccctgataataaagaagaaaggtctattgctatttatctgggaattggcctctgcttgctcttcatcgtccgcacccttctgctgcaccctgccatttttggccttcaccacatcggcatgcaaatgagaattgccatgttctccctcatttacaaaaagaccctgaaactttcctcaagagtgttagataaaatatccattggtcagctggtcagcctgctgtccaacaatcttaacaaatttgatgaaggcttggcgctggcccacttcgtgtggattgcacctctgcaggtggccctgttgatgggacttatatgggagctgcttcaagcctctgctttctgtgggctgggctttttgattgtactggcactttttcaggctgggctcggaagaatgatgatgaaatacagagatcagcgggccgggaagatttcagagcgacttgtgatcaccagtgaaatgattgaaaatattcagagcgtgaaagcctactgctgggaagaagccatggagaagatgattgagaacctgaggcagacagagctcaagctcactcggaaggctgcttatgttcgctatttcaacagcagcgccttcttcttcagtggcttctttgttgtcttcctgtctgttctgccatatgcactgataaaaggcattattttacgaaagatcttcaccaccatcagtttttgcatcgttctcaggatggccgtcacaagacagttcccctgggctgtgcagacctggtacgattccttgggggccatcaacaagattcaagatttcttgcaaaaacaagaatataaaactttagaatacaacctcaccaccactgaagtggtcatggaaaatgtgacagccttttgggaggagggttttggagaattgttcgagaaggcaaagcagaataacaacaacaggaagacgagcaatggggacgactctctcttcttcagcaacttttcactgctcgggacccctgtgttgaaagatataaacttcaagatcgagaggggccagctcttggctgtggcaggctccactggagctggtaaaacatctcttctcatggtgatcatgggggaactggagccttccgaaggaaaaatcaagcacagtgggagaatctcattctgcagccagttttcctggatcatgcccggcaccattaaggaaaacatcatatttggagtgtcctatgatgagtaccgctaccggtcagtcatcaaagcctgtcagttggaggaggacatctccaagtttgcagagaaagacaacattgtgcttggagaggggggtatcactctttctggaggacaaagagccaggatctctttggcccgggcagtctacaaggatgcagacctctacttgttggacagtcccttcggctacctcgacgtgctgactgaaaaagaaatttttgaaagctgtgtgtgcaaactgatggcaaacaagaccaggattcttgtcaccagcaagatggaacatctgaagaaagcggacaaaattctgattctgcatgaagggagctcctacttctatggaacatttagcgagcttcagaacctacagccagacttctcctccaaattaatgggctgtgactccttcgaccagttctctgcagaaagaagaaactctatactcacagagaccctccaccgcttctcccttgagggagatgccccagtttcttggacagaaaccaagaagcagtcctttaagcagactggcgagtttggtgaaaagaggaaaaattcaattctcaatccaattaacagtattcgcaagttcagcattgtccagaagacacccctccagatgaatggcatcgaagaagatagtgacgagccgctggagagacggctgagtctggtgccagattcagaacagggggaggccatcctgccccggatcagcgtcatttccacaggccccacattacaagcacggcgccggcagagtgttttaaatctcatgacccattcagtgaaccagggccaaaatatccacaggaagactacagcttctacccggaaagtgtctctggcccctcaggccaatctgaccgagctggacatctacagcaggaggctctcccaggaaacagggctggaaatatctgaagagattaatgaagaggatcttaaagagtgcttctttgatgacatggagagcatccccgcggtgaccacatggaacacctaccttagatatattactgtccacaagagcctcatatttgtcctcatctggtgcctggttattttcctcgctgaggtggcggccagtcttgttgtgctctggctgctgggcaacactcctctccaggacaagggcaatagtactcacagcagaaataattcttatgccgtcatcattacaagcacctccagctactacgtgttctacatctatgtgggcgtggctgacaccctcctggccatgggtttcttccggggcctgcctttggtgcacaccctcatcacagtgtcaaaaattctgcaccataaaatgcttcattctgtcctgcaggcacccatgagcactttgaacacattgaaggctggcggcatcctcaacagattttctaaagatattgctatcctggatgatctcctccccctgacaatctttgactttatccagcttctgctgatcgtgattggagccatagcagtggttgctgtcctgcagccctacatttttgtggccaccgtgcccgtgattgttgcctttattatgctcagagcttacttcctgcaaacttctcaacagctcaaacagctagaatctgagggccggagccccatttttacccacctggtgacttccctgaagggactgtggactctgagagcattcgggcgacagccttactttgagacactgttccacaaggccctgaacttgcacactgccaactggtttctttacctgagcacactccgctggttccagatgcggatagagatgatcttcgtcatcttttttatagctgtaaccttcatttctatccttacaacaggagaaggagagggcagggtgggaatcatcctcacgctggctatgaacataatgtccaccttgcagtgggccgtgaattccagtatagatgtggattctctaatgaggagtgtctcccgggtgtttaaattcattgatatgccaactgaggggaaacccaccaagtcaacaaaaccttataagaatggacagctgagcaaggtgatgataattgagaacagccacgtgaagaaggatgacatttggcccagcgggggccagatgactgtgaaggacctgacggccaagtacaccgaaggtggaaatgccattttggaaaacatcagcttctcaatctctcctgggcagagagttggattgctgggtcgcacgggcagcggcaaatcaaccctgctcagtgccttccttcggctcctgaatacagaaggcgaaatccaaattgacggggtgagctgggacagcatcaccctgcagcagtggagaaaagcatttggggtcattccacagaaagttttcatcttctctggcactttcagaaagaacctggacccctatgagcagtggagcgaccaggagatctggaaggttgcagatgaagttggcctgcggagtgtgatagaacaatttcctggcaagctggattttgtgctggtagatggaggctgcgtgctgtcccacggccacaaacagctgatgtgcctcgcccgctccgttctttcaaaggccaaaatcttgcttttggatgagcccagtgctcacctcgacccagtgacctatcagataatccgcaggaccttaaagcaagcttttgccgactgcaccgtcatactgtgtgagcaccggattgaagcaatgctggaatgccagcagtttctggtgatcgaggagaataaggtccggcagtacgacagcatccagaagttgttgaatgagcgcagccttttccgccaggccatctccccatctgacagagtcaagctgtttccacataggaactcctctaagtgcaagtccaagccccagatcgctgccctcaaggaggaaactgaggaagaggtgcaggatacccgcctgtga

SEQ ID NO: 14 - DNA, 4443 bp, Artificial Sequence
  Synthetic polynucleotide
atgcagaggagcccactggagaaagcctccgtggtgagtaaactcttttttagttggaccagacccatcctgcgaaaaggatacaggcagcgcctcgagttgtctgatatctaccagattccttctgtggactcagctgacaatttgagtgagaagctggagcgggagtgggatagagagctggcgagcaaaaaaaaccccaagcttatcaatgctctgcgccgctgctttttctggaggttcatgttttatgggatcttcctgtacctgggggaggtcaccaaagctgttcagccgctccttcttggccgcatcatcgccagctatgaccctgataataaagaagaaaggtctattgctatttatctgggaattggcctctgcttgctcttcatcgtccgcacccttctgctgcaccctgccatttttggccttcaccacatcggcatgcaaatgagaattgccatgttctccctcatttacaaaaagaccctgaaactttcctcaagagtgttagataaaatatccattggtcagctggtcagcctgctgtccaacaatcttaacaaatttgatgaaggcttggcgctggcccacttcgtgtggattgcacctctgcaggtggccctgttgatgggacttatatgggagctgcttcaagcctctgctttctgtgggctgggctttttgattgtactggcactttttcaggctgggctcggaagaatgatgatgaaatacagagatcagcgggccgggaagatatcagagcgacttgtgatcaccagtgaaatgattgaaaatattcagagcgtgaaagcctactgctgggaagaagccatggagaagatgattgagaacctgaggcagacagagctcaagctcactcggaaggctgcttatgttcgctatttcaacagcagcgccttcttcttcagtggcttctttgttgtcttcctgtctgttctgccatatgcactgataaaaggcattattttacgaaagatcttcaccaccatcagtttttgcatcgttctcaggatggccgtcacaagacagttcccctgggctgtgcagacctggtacgattccttgggggccatcaacaagattcaagatttcttgcaaaaacaagaatataaaactttagaatacaacctcaccaccactgaagtggtcatggaaaatgtgacagccttttgggaggagggttttggagaattgttcgagaaggcaaagcagaataacaacaacaggaagacgagcaatggggacgactctctcttcttcagcaacttttcactgctcgggacccctgtgttgaaagatataaacttcaagatcgagaggggccagctcttggctgtggcaggctccactggagctggtaaaacatctcttctcatggtgatcatgggggaactggagccttccgaaggaaaaatcaagcacagtgggagaatctcattctgcagccagttttcctggatcatgcccggcaccattaaggaaaacatcatatttggagtgtcctatgatgagtaccgctaccggtccgtcatcaaagcctgtcagttggaggaggacatctccaagtttgcagagaaagacaacattgtgcttggagaggggggtatcactctttctggaggacaaagagccaggatctctttggcccgggcagtctacaaggatgcagacctctacttgttggacagtcccttcggctacctcgacgtgctgactgaaaaagaaatttttgaaagctgtgtgtgcaaactgatggcaaacaagaccaggattcttgtcaccagcaagatggaacatctgaagaaagcggacaaaattctgattctgcatgaagggagctcctacttctatggaacatttagcgagcttcagaacctacagccagacttctcctccaaattaatgggctgtgactccttcgaccagttctctgcagaaagaagaaactctatactcacagagaccctccaccgcttctcccttgagggagatgccccagtttcttggacagaaaccaagaagcagtcctttaagcagactggcgagtttggtgaaaagaggaaaaattcaattctcaatccaattaacagtattcgcaagttcagcattgtccagaagacacccctccagatgaatggcatcgaagaagatagtgacgagccgctggagagacggctgagtctggtgccagattcagaacagggggaggccatcctgccccggatcagcgtcatttccacaggccccacattacaagcacggcgccggcagagtgttttaaatctcatgacccattcagtgaaccagggccaaaatatccacaggaagactacagcttctacccggaaagtgtctctggcccctcaggccaatctgaccgagctggacatctacagcaggaggctctcccaggaaacagggcttgaaatatctgaagagattaatgaagaggatcttaaagagtgcttctttgatgacatggagagcatccccgcggtgaccacatggaacacctaccttagatatattactgtccacaagagcctcatatttgtcctcatctggtgcctggttattttcctcgctgaggtggcggccagtcttgttgtgctctggctgctgggcaacactcctctccaggacaagggcaatagtactcacagcagaaataattcttatgccgtcatcattacaagcacctccagctactacgtgttctacatctatgtgggcgtggctgacaccctcctggccatgggtttcttccggggcctgcctttggtgcacaccctcatcacagtgtcaaaaattctgcaccataaaatgcttcattctgtcctgcaggcacccatgagcactttgaacacattgaaggctggcggcatcctcaacagattttctaaagatattgctatcctggatgatctcctccccctgacaatctttgactttatccagcttctgctgatcgtgattggagccatagcagtggttgctgtcctgcagccctacatttttgtggccaccgtgcccgtgattgttgcctttattatgctcagagcttacttcctgcaaacttctcaacagctcaaacagctagaatctgagggccggagccccatttttacccacctggtgacttccctgaagggactgtggactctgagagcattcgggcgacagccttactttgagacactgttccacaaggccctgaacttgcacactgccaactggtttctttacctgagcacactccgctggttccagatgcggatagagatgatcttcgtcatcttttttatagctgtaaccttcatttctatccttacaacaggagaaggagagggcagggtgggaatcatcctcacgctggctatgaacataatgtccaccttgcagtgggccgtgaattccagtatagatgtggattctctaatgaggagtgtctcccgggtgtttaaattcattgatatgcctactgaggggaaacccaccaagtcaacaaagccttataagaatggacagctgagcaaggtgatgataattgagaacagccacgtgaagaaggatgacatttggcccagcgggggccagatgactgtgaaggacctgacggccaagtacaccgaaggtggaaatgccattttggaaaacatcagcttctcaatctctcctgggcagagagttggattgctgggtcgcacgggcagcggcaaatcaaccctgctcagtgccttccttcggctcctgaatacagaaggcgaaatccaaattgacggggtgagctgggacagcatcaccctgcagcagtggagaaaagcatttggggtcattccacagaaagttttcatcttctctggcactttcagaaagaacctggacccctatgagcagtggagcgaccaggagatctggaaggttgcagatgaagttggcctgcggagtgtgatagaacaatttcctggcaagctggattttgtgctggtagatggaggctgcgtgctgtcccacggccacaaacagctgatgtgcctcgcccgctccgttctttcaaaggccaaaatcttgcttttggatgagcccagtgctcacctcgacccagtgacctatcagataatccgcaggaccttaaagcaagcttttgccgactgcaccgtcatactgtgtgagcaccggattgaagcaatgctggaatgccagcagtttctggtgatcgaggagaataaggtccggcagtacgacagcatccagaagttgttgaatgagcgcagccttttccgccaggccatctccccatctgacagagtcaagctgtttccacataggaactcctctaagtgcaagtccaagccccagatcgctgccctcaaggaggaaactgaggaagaggtgcaggatacccgcctgtga

SEQ ID NO: 15 - DNA, 4443 bp, Artificial Sequence
  Synthetic polynucleotide
atgcagaggagcccactggagaaagcctccgtggtgagtaaactcttttttagttggaccagacccatcctgcgaaaaggatacaggcagcgcctcgagttgtcagatatctaccagattccttctgtggactcagctgacaatttgagtgagaagctggagcgggagtgggatagagagctggcgagcaaaaaaaaccccaagcttatcaatgctctgcgccgctgctttttctggaggttcatgttttatgggatcttcctgtacctgggggaggtcaccaaagctgttcagccgctccttcttggccgcatcatcgccagctatgaccctgataataaagaagaaaggtctattgctatttatctgggaattggcctctgcttgctcttcatcgtccgcacccttctgctgcaccctgccatttttggccttcaccacatcggcatgcaaatgagaattgccatgttctccctcatttacaaaaagaccctgaaactttcctcaagagtgttagataaaatatccattggtcagctggtcagcctgctgtccaacaatcttaacaaatttgatgaaggcttggcgctggcccacttcgtgtggattgcacctctgcaggtggccctgttgatgggacttatatgggagctgcttcaagcctctgctttctgtgggctgggctttttgattgtactggcactttttcaggctgggctcggaagaatgatgatgaaatacagagatcagcgggccgggaagatatcagagcgacttgtgatcaccagtgaaatgattgaaaatattcagagcgtgaaagcctactgctgggaagaagccatggagaagatgattgagaacctgaggcagacagagctcaagctcactcggaaggctgcttatgttcgctatttcaacagcagcgccttcttcttcagtggcttctttgttgtcttcctgtctgttctgccatatgcactgataaaaggcattattttacgaaagatcttcaccaccatcagtttttgcatcgttctcaggatggccgtcacaagacagttcccctgggctgtgcagacctggtacgattccttgggggccatcaacaagattcaagatttcttgcaaaaacaagaatataaaactttagaatacaacctcaccaccactgaagtggtcatggaaaatgtgacagccttttgggaggagggttttggagaattgttcgagaaggcaaagcagaataacaacaacaggaagacgagcaatggggacgactctctcttcttcagcaacttttcactgctcgggacccctgtgttgaaagatataaacttcaagatcgagaggggccagctcttggctgtggcaggctccactggagctggtaaaacatctcttctcatggtgatcatgggggaactggagccttccgaaggaaaaatcaagcacagtgggagaatctcattctgcagccagttttcctggatcatgcccggcaccattaaggaaaacatcatatttggagtgtcctatgatgagtaccgctaccggtcagtcatcaaagcctgtcagttggaggaggacatctccaagtttgcagagaaagacaacattgtgcttggagaggggggtatcactctttctggaggacaaagagccaggatctctttggcccgggcagtctacaaggatgcagacctctacttgttggacagtcccttcggctacctcgacgtgctgactgaaaaagaaatttttgaaagctgtgtgtgcaaactgatggcaaacaagaccaggattcttgtcaccagcaagatggaacatctgaagaaagcggacaaaattctgattctgcatgaagggagctcctacttctatggaacatttagcgagcttcagaacctacagccagacttctcctccaaattaatgggctgtgactccttcgaccagttctctgcagaaagaagaaactctatactcacagagaccctccaccgcttctcccttgagggagatgccccagtttcttggacagaaaccaagaagcagtcctttaagcagactggcgagtttggtgaaaagaggaaaaattcaattctcaatcctattaacagtattcgcaagttcagcattgtccagaagacacccctccagatgaatggcatcgaagaagatagtgacgagccgctggagagacggctgagtctggtgccagattcagaacagggggaggccatcctgccccggatcagcgtcatttccacaggccccacattacaagcacggcgccggcagagtgttttaaatctcatgacccattcagtgaaccagggccaaaatatccacaggaagactacagcttctacccggaaagtgtctctggcccctcaggccaatctgaccgagctggacatctacagcaggaggctctcccaggaaacagggcttgaaatatctgaagagattaatgaagaggatcttaaagagtgcttctttgatgacatggagagcatccccgcggtgaccacatggaacacctaccttagatatattactgtccacaagagcctcatatttgtcctcatctggtgcctggttattttcctcgctgaggtggcggccagtcttgttgtgctctggctgctgggcaacactcctctccaggacaagggcaatagtacacacagcagaaataattcttatgccgtcatcattacaagcacctccagctactacgtgttctacatctatgtgggcgtggctgacaccctcctggccatgggtttcttccggggcctgcctttggtgcacaccctcatcacagtgtcaaaaattctgcaccataaaatgcttcattctgtcctgcaggcacccatgagcactttgaacacattgaaggctggcggcatcctcaacagattttctaaagatattgctatcctggatgatctcctccccctgacaatctttgactttatccagcttctgctgatcgtgattggagccatagcagtggttgctgtcctgcagccctacatttttgtggccaccgtgcccgtgattgttgcctttattatgctcagagcttacttcctgcaaacttctcaacagctcaaacagctagaatctgagggccggagccccatttttacccacctggtgacttccctgaagggactgtggactctgagagcattcgggcgacagccttactttgagacactgttccacaaggccctgaacttgcacactgccaactggtttctttacctgagcacactccgctggttccagatgcggatagagatgatcttcgtcatcttttttatagctgtaaccttcatttctatccttacaacaggagaaggagagggcagggtgggaatcatcctcacgctggctatgaacataatgtccaccttgcagtgggccgtgaattccagtatagatgtggattctctaatgaggagtgtctcccgggtgtttaaattcattgatatgcctactgaggggaaacccaccaagtcaacaaaaccttataagaatggacagctgagcaaggtgatgataattgagaacagccacgtgaagaaggatgacatttggcccagcgggggccagatgactgtgaaggacctgacggccaagtacaccgaaggtggaaatgccattttggaaaacatcagcttctcaatctctcctgggcagagagttggattgctgggtcgcacgggcagcggcaaatcaaccctgctcagtgccttccttcggctcctgaatacagaaggcgaaatccaaattgacggggtgagctgggacagcatcaccctgcagcagtggagaaaagcatttggggtcattccacagaaagttttcatcttctctggcactttcagaaagaacctggacccctatgagcagtggagcgaccaggagatctggaaggttgcagatgaagttggcctgcggagtgtgatagaacaatttcctggcaagctggattttgtgctggtagatggaggctgcgtgctgtcccacggccacaaacagctgatgtgcctcgcccgctccgttctttcaaaggccaaaatcttgcttttggatgagcccagtgctcacctcgacccagtgacctatcagataatccgcaggaccttaaagcaagcttttgccgactgcaccgtcatactgtgtgagcaccggattgaagcaatgctggaatgccagcagtttctggtgatcgaggagaataaggtccggcagtacgacagcatccagaagttgttgaatgagcgcagccttttccgccaggccatctccccatctgacagagtcaagctgtttccacataggaactcctctaagtgcaagtccaagccccagatcgctgccctcaaggaggaaactgaggaagaggtgcaggatacccgcctgtga

SEQ ID NO: 16 - DNA, 4443 bp, Artificial Sequence
  Synthetic polynucleotide
atgcagaggagcccactggagaaagcctccgtggtgagtaaactcttttttagttggaccagacccatcctgcgaaaaggatacaggcagcgcctcgagttgtcagatatctaccagattccttctgtggactcagctgacaatttgagtgagaagctggagcgggagtgggatagagagctggcgagcaaaaaaaaccccaagcttatcaatgctctgcgccgctgctttttctggaggttcatgttttatgggatcttcctgtacctgggggaggtcaccaaagctgttcagccgctccttcttggccgcatcatcgccagctatgaccctgataataaagaagaaaggtctattgctatttatctgggaattggcctctgcttgctcttcatcgtccgcacccttctgctgcaccctgccatttttggccttcaccacatcggcatgcaaatgagaattgccatgttctccctcatttacaaaaagaccctgaaactttcctcaagagtgttagataaaatatccattggtcagctggtcagcctgctgtccaacaatcttaacaaatttgatgaaggcttggcgctggcccacttcgtgtggattgcacctctgcaggtggccctgttgatgggacttatatgggagctgcttcaagcctctgctttctgtgggctgggctttttgattgtactggcactttttcaggctgggctcggaagaatgatgatgaaatacagagatcagcgggccgggaagatatcagagcgacttgtgatcaccagtgaaatgattgaaaatattcagagcgtgaaagcctactgctgggaagaagccatggagaagatgattgagaacctgaggcagacagagctcaagctcactcggaaggctgcttatgttcgctatttcaacagcagcgccttcttcttcagtggcttctttgttgtcttcctgtctgttctgccatatgcactgataaaaggcattattttacgaaagatcttcaccaccatcagtttttgcatcgttctcaggatggccgtcacaagacagttcccctgggctgtgcagacctggtacgattccttgggggccatcaacaagattcaagatttcttgcaaaaacaagaatataaaactttagaatacaacctcaccaccactgaagtggtcatggaaaatgtgacagccttttgggaggagggttttggagaattgttcgagaaggcaaagcagaataacaacaacaggaagacgagcaatggggacgactctctcttcttcagcaacttttcactgctcgggacccctgtgttgaaagatataaacttcaagatcgagaggggccagctcttggctgtggcaggctccactggagctggtaaaacatctcttctcatggtgatcatgggggaactggagccttccgaaggaaaaatcaagcacagtgggagaatctcattctgcagccagttttcctggatcatgcccggcaccattaaggaaaacatcatatttggagtgtcctatgatgagtaccgctaccggtccgtcatcaaagcctgtcagttggaggaggacatctccaagtttgcagagaaagacaacattgtgcttggagaggggggtatcactctttctggaggacaaagagccaggatctctttggcccgggcagtctacaaggatgcagacctctacttgttggacagtcccttcggctacctcgacgtgctgactgaaaaagaaatttttgaaagctgtgtgtgcaaactgatggcaaacaagaccaggattcttgtcaccagcaagatggaacatctgaagaaagcggacaaaattctgattctgcatgaagggagctcctacttctatggaacatttagcgagcttcagaacctacagccagacttctcctccaaattaatgggctgtgactccttcgaccagttctctgcagaaagaagaaactctatactcacagagaccctccaccgcttctcccttgagggagatgccccagtttcttggacagaaaccaagaagcagtcctttaagcagactggcgagtttggtgaaaagaggaaaaattcaattctcaatccaattaacagtattcgcaagttcagcattgtccagaagacacccctccagatgaatggcatcgaagaagatagtgacgagccgctggagagacggctgagtctggtgccagattcagaacagggggaggccatcctgccccggatcagcgtcatttccacaggccccacattacaagcacggcgccggcagagtgttttaaatctcatgacccattcagtgaaccagggccaaaatatccacaggaagactacagcttctacccggaaagtgtctctggcccctcaggccaatctgaccgagctggacatctacagcaggaggctctcccaggaaacagggctggaaatatctgaagagattaatgaagaggatcttaaagagtgcttctttgatgacatggagagcatccccgcggtgaccacatggaacacctaccttagatatattactgtccacaagagcctcatatttgtcctcatctggtgcctggttattttcctcgctgaggtggcggccagtcttgttgtgctctggctgctgggcaacactcctctccaggacaagggcaatagtactcacagcagaaataattcttatgccgtcatcattacaagcacctccagctactacgtgttctacatctatgtgggcgtggctgacaccctcctggccatgggtttcttccggggcctgcctttggtgcacaccctcatcacagtgtcaaaaattctgcaccataaaatgcttcattctgtcctgcaggcacccatgagcactttgaacacattgaaggctggcggcatcctcaacagattttctaaagatattgctatcctggatgatctcctccccctgacaatctttgactttatccagcttctgctgatcgtgattggagccatagcagtggttgctgtcctgcagccctacatttttgtggccaccgtgcccgtgattgttgcctttattatgctcagagcttacttcctgcaaacttctcaacagctcaaacagctagagtctgagggccggagccccatttttacccacctggtgacttccctgaagggactgtggactctgagagcattcgggcgacagccttactttgagacactgttccacaaggccctgaacttgcacactgccaactggtttctttacctgagcacactccgctggttccagatgcggatagagatgatcttcgtcatcttttttatagctgtaaccttcatttctatccttacaacaggagaaggagagggcagggtgggaatcatcctcacgctggctatgaacataatgtccaccttgcagtgggccgtgaattccagtatagatgtggattctctaatgaggagtgtctcccgggtgtttaaattcattgatatgcctactgaggggaaacccaccaagtcaacaaaaccttataagaatggacagctgagcaaggtgatgataattgagaacagccacgtgaagaaggatgacatttggcccagcgggggccagatgactgtgaaggacctgacggccaagtacaccgaaggtggaaatgccattttggaaaacatcagcttctcaatctctcctgggcagagagttggattgctgggtcgcacgggcagcggcaaatcaaccctgctcagtgccttccttcggctcctgaatacagaaggcgaaatccaaattgacggggtgagctgggacagcatcaccctgcagcagtggagaaaagcatttggggtcattccacagaaagttttcatcttctctggcactttcagaaagaacctggacccctatgagcagtggagcgaccaggagatctggaaggttgcagatgaagttggcctgcggagtgtgatagaacaatttcctggcaagctggattttgtgctggtagatggaggctgcgtgctgtcccacggccacaaacagctgatgtgcctcgcccgctccgttctttcaaaggccaaaatcttgcttttggatgagcccagtgctcacctcgacccagtgacctatcagataatccgcaggaccttaaagcaagcttttgccgactgcaccgtcatactgtgtgagcaccggattgaagcaatgctggaatgccagcagtttctggtgatcgaggagaataaggtccggcagtacgacagcatccagaagttgttgaatgagcgcagccttttccgccaggccatctccccatctgacagagtcaagctgtttccacataggaactcctctaagtgcaagtccaagccccagatcgctgccctcaaggaggaaactgaggaagaggtgcaggatacccgcctgtga

SEQ ID NO: 17 - DNA, 4443 bp, Artificial Sequence
  Synthetic polynucleotide
atgcagaggagcccactggagaaagcctccgtggtgagtaaactcttttttagttggaccagacccatcctgcgaaaaggatacaggcagcgcctcgagttgtctgatatctaccagattccttctgtggactcagctgacaatttgagtgagaagctggagcgggagtgggatagagagctggcgagcaaaaaaaaccccaagcttatcaatgctctgcgccgctgctttttctggaggttcatgttttatgggatcttcctgtacctgggggaggtcaccaaagctgttcagccgctccttcttggccgcatcatcgccagctatgaccctgataataaagaagaaaggtctattgctatttatctgggaattggcctctgcttgctcttcatcgtccgcacccttctgctgcaccctgccatttttggccttcaccacatcggcatgcaaatgagaattgccatgttctccctcatttacaaaaagaccctgaaactttcctcaagagtgttagataaaatatccattggtcagctggtcagcctgctgtccaacaatcttaacaaatttgatgaaggcttggcgctggcccacttcgtgtggattgcacctctgcaggtggccctgttgatgggacttatatgggagctgcttcaagcctctgctttctgtgggctgggctttttgattgtactggcactttttcaggctgggctcggaagaatgatgatgaaatacagagatcagcgggccgggaagatttcagagcgacttgtgatcaccagtgaaatgattgaaaatattcagagcgtgaaagcctactgctgggaagaagccatggagaagatgattgagaacctgaggcagacagagctcaagctcactcggaaggctgcttatgttcgctatttcaacagcagcgccttcttcttcagtggcttctttgttgtcttcctgtctgttctgccatatgcactgataaaaggcattattttacgaaagatcttcaccaccatcagtttttgcatcgttctcaggatggccgtcacaagacagttcccctgggctgtgcagacctggtacgattccttgggggccatcaacaagattcaagatttcttgcaaaaacaagaatataaaactttagaatacaacctcaccaccactgaagtggtcatggaaaatgtgacagccttttgggaggagggttttggagaattgttcgagaaggcaaagcagaataacaacaacaggaagacgagcaatggggacgactctctcttcttcagcaacttttcactgctcgggacccctgtgttgaaagatataaacttcaagatcgagaggggccagctcttggctgtggcaggctccactggagctggtaaaacatctcttctcatggtgatcatgggggaactggagccttccgaaggaaaaatcaagcacagtgggagaatctcattctgcagccagttttcctggatcatgcccggcaccattaaggaaaacatcatatttggagtgtcctatgatgagtaccgctaccggtcagtcatcaaagcctgtcagttggaggaggacatctccaagtttgcagagaaagacaacattgtgcttggagaggggggtatcactctttctggaggacaaagagccaggatctctttggcccgggcagtctacaaggatgcagacctctacttgttggacagtcccttcggctacctcgacgtgctgactgaaaaagaaatttttgaaagctgtgtgtgcaaactgatggcaaacaagaccaggattcttgtcaccagcaagatggaacatctgaagaaagcggacaaaattctgattctgcatgaagggagctcctacttctatggaacatttagcgagcttcagaacctacagccagacttctcctccaaattaatgggctgtgactccttcgaccagttctctgcagaaagaagaaactctatactcacagagaccctccaccgcttctcccttgagggagatgccccagtttcttggacagaaaccaagaagcagtcctttaagcagactggcgagtttggtgaaaagaggaaaaattcaattctcaatcctattaacagtattcgcaagttcagcattgtccagaagacacccctccagatgaatggcatcgaagaagatagtgacgagccgctggagagacggctgagtctggtgccagattcagaacagggggaggccatcctgccccggatcagcgtcatttccacaggccccacattacaagcacggcgccggcagagtgttttaaatctcatgacccattcagtgaaccagggccaaaatatccacaggaagactacagcttctacccggaaagtgtctctggcccctcaggccaatctgaccgagctggacatctacagcaggaggctctcccaggaaacagggctggaaatatctgaagagattaatgaagaggatcttaaagagtgcttctttgatgacatggagagcatccccgcggtgaccacatggaacacctaccttagatatattactgtccacaagagcctcatatttgtcctcatctggtgcctggttattttcctcgctgaggtggcggccagtcttgttgtgctctggctgctgggcaacactcctctccaggacaagggcaatagtacacacagcagaaataattcttatgccgtcatcattacaagcacctccagctactacgtgttctacatctatgtgggcgtggctgacaccctcctggccatgggtttcttccggggcctgcctttggtgcacaccctcatcacagtgtcaaaaattctgcaccataaaatgcttcattctgtcctgcaggcacccatgagcactttgaacacattgaaggctggcggcatcctcaacagattttctaaagatattgctatcctggatgatctcctccccctgacaatctttgactttatccagcttctgctgatcgtgattggagccatagcagtggttgctgtcctgcagccctacatttttgtggccaccgtgcccgtgattgttgcctttattatgctcagagcttacttcctgcaaacttctcaacagctcaaacagctagaatctgagggccggagccccatttttacccacctggtgacttccctgaagggactgtggactctgagagcattcgggcgacagccttactttgagacactgttccacaaggccctgaacttgcacactgccaactggtttctttacctgagcacactccgctggttccagatgcggatagagatgatcttcgtcatcttttttatagctgtaaccttcatttctatccttacaacaggagaaggagagggcagggtgggaatcatcctcacgctggctatgaacataatgtccaccttgcagtgggccgtgaattccagtatagatgtggattctctaatgaggagtgtctcccgggtgtttaaattcattgatatgcctactgaggggaaacccaccaagtcaacaaaaccttataagaatggacagctgagcaaggtgatgataattgagaacagccacgtgaagaaggatgacatttggcccagcgggggccagatgactgtgaaggacctgacggccaagtacaccgaaggtggaaatgccattttggaaaacatcagcttctcaatctctcctgggcagagagttggattgctgggtcgcacgggcagcggcaaatcaaccctgctcagtgccttccttcggctcctgaatacagaaggcgaaatccaaattgacggggtgagctgggacagcatcaccctgcagcagtggagaaaagcatttggggtcattccacagaaagttttcatcttctctggcactttcagaaagaacctggacccctatgagcagtggagcgaccaggagatctggaaggttgcagatgaagttggcctgcggagtgtgatagaacaatttcctggcaagctggattttgtgctggtagatggaggctgcgtgctgtcccacggccacaaacagctgatgtgcctcgcccgctccgttctttcaaaggccaaaatcttgcttttggatgagcccagtgctcacctcgacccagtgacctatcagataatccgcaggaccttaaagcaagcttttgccgactgcaccgtcatactgtgtgagcaccggattgaagcaatgctggaatgccagcagtttctggtgatcgaggagaataaggtccggcagtacgacagcatccagaagttgttgaatgagcgcagccttttccgccaggccatctccccatctgacagagtcaagctgtttccacataggaactcctctaagtgcaagtccaagccccagatcgctgccctcaaggaggaaactgaggaagaggtgcaggatacccgcctgtga

SEQ ID NO: 18 - DNA, 4443 bp, Artificial Sequence
  Synthetic polynucleotide
atgcagagaagccccctggagaaggcctctgtggtgagcaagctgttcttcagctggaccagacccatcctgagaaagggctacagacagagactggagctgtctgacatctaccagatcccctctgtggactctgccgacaacctgtctgagaagctggagagagagtgggacagagagctggccagcaagaagaaccccaagctgatcaatgccctgagaagatgcttcttctggagattcatgttctatggcatcttcctgtacctgggagaggtgaccaaggccgtgcagcccctgctgctgggcaggatcattgccagctatgaccctgacaacaaggaggagagaagcattgccatctacctgggcattggcctgtgcctgctgttcattgtgagaaccctgctgctgcaccctgccatctttggcctgcaccacattggcatgcagatgagaattgccatgttcagcctgatctacaagaagaccctgaagctgagcagcagagtgctggacaagatcagcattggccagctggtgagcctgctgagcaacaacctgaacaagtttgatgagggcctggccctggcccactttgtgtggattgcccccctgcaggtggccctgctgatgggcctgatctgggagctgctgcaggcctctgccttctgtggcctgggcttcctgattgtgctggccctgttccaggccggcctgggcagaatgatgatgaagtacagagaccagagagccggcaagatctctgagagactggtgatcacctctgagatgattgagaacatccagtctgtgaaggcctactgctgggaggaggccatggagaagatgattgagaacctgagacagacagagctgaagctgaccaggaaggccgcctatgtgagatacttcaacagctctgccttcttcttctctggcttctttgtggtgttcctgtctgtgctgccctatgccctgatcaagggcatcatcctgaggaagatcttcaccaccatcagcttctgcattgtgctgaggatggccgtgaccaggcagttcccctgggccgtgcagacctggtatgacagcctgggggccatcaacaagatccaggacttcctgcagaagcaggagtacaagaccctggagtacaacctgaccaccacagaggtggtgatggagaatgtgacagccttctgggaggagggctttggagagctgtttgagaaggccaagcagaacaacaacaacagaaagaccagcaatggagatgacagcctgttcttcagcaacttcagcctgctgggcacccctgtgctgaaggacatcaacttcaagattgagaggggccagctgctggccgtggccggcagcacaggagccggcaagaccagcctgctgatggtgatcatgggagagctggagccctctgagggcaagatcaagcactctggcagaatcagcttctgcagccagttcagctggatcatgcctggcaccatcaaggagaacatcatctttggggtgagctatgatgagtacaggtacagatctgtgatcaaggcctgccagctggaggaggacatctccaagtttgccgagaaggacaacattgtgctgggggagggaggcatcaccctgtctgggggccagagagccagaatcagcctggccagagccgtgtacaaggatgccgacctgtacctgctggacagcccctttggctacctggatgtgctgacagagaaggagatctttgagagctgtgtgtgcaagctgatggccaacaagaccaggatcctggtgaccagcaagatggagcacctgaagaaggccgacaagatcctgatcctgcatgagggcagcagctacttctatggcaccttctctgagctgcagaacctgcagcctgacttcagcagcaagctgatgggctgtgacagctttgaccagttctctgctgagagaagaaacagcatcctgacagagaccctgcacaggttcagcctggagggggatgcccctgtgagctggacagagaccaagaagcagagcttcaagcagacaggagagtttggggagaagaggaagaacagcatcctgaaccccatcaacagcatcaggaagttcagcattgtgcagaagacccccctgcagatgaatggcattgaggaggactctgatgagcccctggagagaagactgagcctggtgccagactctgagcagggagaggccatcctgcccaggatctctgtgatcagcacaggccccaccctgcaggccagaagaagacagtctgtgctgaacctgatgacccactctgtgaaccagggccagaatatccacagaaagaccacagccagcaccagaaaggtgagcctggccccccaggccaacctgacagagctggacatctacagcagaaggctgagccaggagacaggcctggagatctctgaggagatcaatgaggaggacctgaaggagtgcttctttgatgacatggagagcatccctgccgtgaccacctggaacacctacctgagatacatcacagtgcacaagagcctgatctttgtgctgatctggtgcctggtgatcttcctggccgaggtggccgccagcctggtggtgctgtggctgctgggcaacacccccctgcaggacaagggcaacagcacccacagcagaaacaacagctatgctgtgatcatcaccagcaccagcagctactatgtgttctacatctatgtgggagtggctgacaccctgctggccatgggcttcttcagaggcctgcccctggtgcacaccctgatcacagtgagcaagatcctgcaccacaagatgctgcactctgtgctgcaggcccccatgagcaccctgaacaccctgaaggctggaggcatcctgaacagattcagcaaggacattgccatcctggatgacctgctgcccctgaccatctttgacttcatccagctgctgctgattgtgattggagccattgccgtggtggccgtgctgcagccctacatctttgtggccacagtgcctgtgattgtggccttcatcatgctgagggcctacttcctgcagaccagccagcagctgaagcagctggagtctgagggcagaagccccatcttcacccacctggtgaccagcctgaagggcctgtggaccctgagggcctttggcagacagccctactttgagaccctgttccacaaggccctgaacctgcacacagccaactggttcctgtacctgagcaccctgagatggttccagatgaggattgagatgatctttgtgatcttcttcattgccgtgaccttcatcagcatcctgaccacaggggagggcgagggcagagtgggcatcatcctgaccctggccatgaacatcatgagcaccctgcagtgggccgtgaacagcagcattgatgtggacagcctgatgagatctgtgagcagagtgttcaagttcattgacatgcccacagagggcaagcccaccaagagcaccaagccctacaagaatggccagctgagcaaggtgatgatcattgagaacagccatgtgaagaaggatgacatctggccctctggaggccagatgacagtgaaggacctgacagccaagtacacagaggggggcaatgccatcctggagaacatcagcttcagcatcagccctggccagagggtgggcctgctgggcagaacaggctctggcaagagcaccctgctgtctgccttcctgaggctgctgaacacagagggagagatccagattgatggggtgagctgggacagcatcaccctgcagcagtggaggaaggcctttggggtgatcccccagaaggtgttcatcttctctggcaccttcaggaagaacctggacccctatgagcagtggtctgaccaggagatctggaaggtggccgatgaggtgggcctgagatctgtgattgagcagttccctggcaagctggactttgtgctggtggatggaggctgtgtgctgagccatggccacaagcagctgatgtgcctggccagatctgtgctgagcaaggccaagatcctgctgctggatgagccctctgcccacctggaccctgtgacctaccagatcatcagaagaaccctgaagcaggcctttgccgactgcacagtgatcctgtgtgagcacagaattgaggccatgctggagtgccagcagttcctggtgattgaggagaacaaggtgaggcagtatgacagcatccagaagctgctgaatgagagaagcctgttcagacaggccatcagcccctctgacagagtgaagctgttcccccacaggaacagcagcaagtgcaagagcaagccccagattgccgccctgaaggaggagacagaggaggaggtgcaggacaccagactgtga

SEQ ID NO: 19 - DNA, 4443 bp, Artificial Sequence
  Synthetic polynucleotide
atgcagaggagccccctggagaaggccagcgtggtgagcaagctgttcttcagctggaccaggcccatcctgaggaagggctacaggcagaggctggagctgagcgacatctaccagatccccagcgtggacagcgccgacaacctgagcgagaagctggagagggagtgggacagggagctggccagcaagaagaaccccaagctgatcaacgccctgaggaggtgcttcttctggaggttcatgttctacggcatcttcctgtacctgggcgaggtgaccaaggccgtgcagcccctgctgctgggcaggatcatcgccagctacgaccccgacaacaaggaggagaggagcatcgccatctacctgggcatcggcctgtgcctgctgttcatcgtgaggaccctgctgctgcaccccgccatcttcggcctgcaccacatcggcatgcagatgaggatcgccatgttcagcctgatctacaagaagaccctgaagctgagcagcagggtgctggacaagatcagcatcggccagctggtgagcctgctgagcaacaacctgaacaagttcgacgagggcctggccctggcccacttcgtgtggatcgcccccctgcaggtggccctgctgatgggcctgatctgggagctgctgcaggccagcgccttctgcggcctgggcttcctgatcgtgctggccctgttccaggccggcctgggcaggatgatgatgaagtacagggaccagagggccggcaagatcagcgagaggctggtgatcaccagcgagatgatcgagaacatccagagcgtgaaggcctactgctgggaggaggccatggagaagatgatcgagaacctgaggcagaccgagctgaagctgaccaggaaggccgcctacgtgaggtacttcaacagcagcgccttcttcttcagcggcttcttcgtggtgttcctgagcgtgctgccctacgccctgatcaagggcatcatcctgaggaagatcttcaccaccatcagcttctgcatcgtgctgaggatggccgtgaccaggcagttcccctgggccgtgcagacctggtacgacagcctgggcgccatcaacaagatccaggacttcctgcagaagcaggagtacaagaccctggagtacaacctgaccaccaccgaggtggtgatggagaacgtgaccgccttctgggaggagggcttcggcgagctgttcgagaaggccaagcagaacaacaacaacaggaagaccagcaacggcgacgacagcctgttcttcagcaacttcagcctgctgggcacccccgtgctgaaggacatcaacttcaagatcgagaggggccagctgctggccgtggccggcagcaccggcgccggcaagaccagcctgctgatggtgatcatgggcgagctggagcccagcgagggcaagatcaagcacagcggcaggatcagcttctgcagccagttcagctggatcatgcccggcaccatcaaggagaacatcatcttcggcgtgagctacgacgagtacaggtacaggagcgtgatcaaggcctgccagctggaggaggacatcagcaagttcgccgagaaggacaacatcgtgctgggcgagggcggcatcaccctgagcggcggccagagggccaggatcagcctggccagggccgtgtacaaggacgccgacctgtacctgctggacagccccttcggctacctggacgtgctgaccgagaaggagatcttcgagagctgcgtgtgcaagctgatggccaacaagaccaggatcctggtgaccagcaagatggagcacctgaagaaggccgacaagatcctgatcctgcacgagggcagcagctacttctacggcaccttcagcgagctgcagaacctgcagcccgacttcagcagcaagctgatgggctgcgacagcttcgaccagttcagcgccgagaggaggaacagcatcctgaccgagaccctgcacaggttcagcctggagggcgacgcccccgtgagctggaccgagaccaagaagcagagcttcaagcagaccggcgagttcggcgagaagaggaagaacagcatcctgaaccccatcaacagcatcaggaagttcagcatcgtgcagaagacccccctgcagatgaacggcatcgaggaggacagcgacgagcccctggagaggaggctgagcctggtgcccgacagcgagcagggcgaggccatcctgcccaggatcagcgtgatcagcaccggccccaccctgcaggccaggaggaggcagagcgtgctgaacctgatgacccacagcgtgaaccagggccagaacatccacaggaagaccaccgccagcaccaggaaggtgagcctggccccccaggccaacctgaccgagctggacatctacagcaggaggctgagccaggagaccggcctggagatcagcgaggagatcaacgaggaggacctgaaggagtgcttcttcgacgacatggagagcatccccgccgtgaccacctggaacacctacctgaggtacatcaccgtgcacaagagcctgatcttcgtgctgatctggtgcctggtgatcttcctggccgaggtggccgccagcctggtggtgctgtggctgctgggcaacacccccctgcaggacaagggcaacagcacccacagcaggaacaacagctacgccgtgatcatcaccagcaccagcagctactacgtgttctacatctacgtgggcgtggccgacaccctgctggccatgggcttcttcaggggcctgcccctggtgcacaccctgatcaccgtgagcaagatcctgcaccacaagatgctgcacagcgtgctgcaggcccccatgagcaccctgaacaccctgaaggccggcggcatcctgaacaggttcagcaaggacatcgccatcctggacgacctgctgcccctgaccatcttcgacttcatccagctgctgctgatcgtgatcggcgccatcgccgtggtggccgtgctgcagccctacatcttcgtggccaccgtgcccgtgatcgtggccttcatcatgctgagggcctacttcctgcagaccagccagcagctgaagcagctggagagcgagggcaggagccccatcttcacccacctggtgaccagcctgaagggcctgtggaccctgagggccttcggcaggcagccctacttcgagaccctgttccacaaggccctgaacctgcacaccgccaactggttcctgtacctgagcaccctgaggtggttccagatgaggatcgagatgatcttcgtgatcttcttcatcgccgtgaccttcatcagcatcctgaccaccggcgagggcgagggcagggtgggcatcatcctgaccctggccatgaacatcatgagcaccctgcagtgggccgtgaacagcagcatcgacgtggacagcctgatgaggagcgtgagcagggtgttcaagttcatcgacatgcccaccgagggcaagcccaccaagagcaccaagccctacaagaacggccagctgagcaaggtgatgatcatcgagaacagccacgtgaagaaggacgacatctggcccagcggcggccagatgaccgtgaaggacctgaccgccaagtacaccgagggcggcaacgccatcctggagaacatcagcttcagcatcagccccggccagagggtgggcctgctgggcaggaccggcagcggcaagagcaccctgctgagcgccttcctgaggctgctgaacaccgagggcgagatccagatcgacggcgtgagctgggacagcatcaccctgcagcagtggaggaaggccttcggcgtgatcccccagaaggtgttcatcttcagcggcaccttcaggaagaacctggacccctacgagcagtggagcgaccaggagatctggaaggtggccgacgaggtgggcctgaggagcgtgatcgagcagttccccggcaagctggacttcgtgctggtggacggcggctgcgtgctgagccacggccacaagcagctgatgtgcctggccaggagcgtgctgagcaaggccaagatcctgctgctggacgagcccagcgcccacctggaccccgtgacctaccagatcatcaggaggaccctgaagcaggccttcgccgactgcaccgtgatcctgtgcgagcacaggatcgaggccatgctggagtgccagcagttcctggtgatcgaggagaacaaggtgaggcagtacgacagcatccagaagctgctgaacgagaggagcctgttcaggcaggccatcagccccagcgacagggtgaagctgttcccccacaggaacagcagcaagtgcaagagcaagccccagatcgccgccctgaaggaggagaccgaggaggaggtgcaggacaccaggctgtga

SEQ ID NO: 20 - DNA, 4443 bp, Artificial Sequence
  Synthetic polynucleotide
atgcagagatcccctctggagaaggcctcagtggtgtccaagcttttcttctcctggaccaggcccattttaagaaagggctacaggcagagacttgagctgtctgacatctatcagatcccttctgtggattctgctgacaatcttagtgaaaaattggaaagggagtgggacagagagctggcaagtaaaaagaaccccaagctgattaatgccctgaggcgctgctttttttggagattcatgttctatggcatattcctctaccttggagaagtaaccaaagctgtacagcctctcctccttggcagaatcattgcctcctatgatcctgataacaaggaggagagaagcatagccatctacctgggcattgggctgtgcctcttgtttattgtgaggacccttctcttgcaccctgccatctttggccttcatcacattggcatgcaaatgagaatagcaatgtttagtcttatttacaaaaaaacattaaaactctcttccagggtgttggacaagatcagtattggacaactggtcagcctgctgagcaacaacctgaacaagtttgatgaaggactggccctggcccactttgtctggattgccccccttcaggtggctcttttgatgggcctgatctgggaactcctgcaggcctctgccttctgtgggttaggcttcctgatagtgctagctctctttcaggcagggttgggtagaatgatgatgaagtacagagaccagagggctgggaagatatctgagaggctggtcattacttctgaaatgatagaaaacatccagtctgttaaagcttactgctgggaggaggctatggaaaagatgattgagaacttgaggcaaacagagctcaagctgactaggaaggcagcctatgtcaggtatttcaacagcagtgctttcttcttctcaggctttttcgtggtcttcttgagtgttctgccctatgccctcatcaaggggataattttgagaaagattttcaccactatttccttttgcattgtcctgaggatggctgtcaccaggcaattcccctgggctgtgcagacatggtatgactctctgggggccatcaacaaaatccaagatttcctgcagaagcaggagtacaagaccctggaatacaacctcaccaccacagaagttgtgatggagaatgtgactgcattctgggaggaaggatttggggagctgtttgagaaagcaaaacaaaacaataataacaggaaaaccagcaatggagatgactccctgttcttttccaacttctctttgttgggcacccctgtcctgaaagatataaactttaaaattgaaagagggcagctgttggcagttgctggctccacaggagctggaaaaacttcactactgatggtgatcatgggggagttagaaccctctgaagggaaaataaaacattctgggaggattagtttctgcagccagttcagctggatcatgcctgggaccattaaagaaaatattatatttggagtgagctatgatgaatatagatataggagtgtcatcaaagcctgtcagttggaggaagacatcagcaaatttgcagagaaagacaacattgttctgggtgaaggtggcatcaccctgtcaggagggcaaagggccaggatcagcttggccagagcagtctataaagatgctgatctgtacctcctggatagcccttttggctatctggatgttttgacagagaaggaaatttttgagtcctgtgtctgcaagttaatggcaaataaaacaaggatacttgtgacctcaaaaatggaacacctgaagaaggctgacaaaattctgatcctgcatgagggcagcagctacttttatggaacattttctgaactgcagaatttgcaaccagacttttcatcaaagctcatgggatgtgacagttttgatcagttttctgcagaaaggagaaactccattttgactgagaccctgcacaggttcagtctggagggggatgccccagtgagttggactgagacaaagaaacagagcttcaagcagactggagagtttggagaaaagaggaaaaactcaattctcaatcccatcaatagcatcaggaagttcagcatagttcagaagactcctttgcagatgaatgggattgaagaggactcagatgagcccctggaaaggagactctccttggtgccagattcagagcagggggaagccatactgccaaggatctctgtgatttctacagggcccaccctccaagcaagaaggagacagtcagttttaaacctgatgacccactctgtcaaccagggacagaacattcatagaaagacaacagcatctacaagaaaagtttcactggcccctcaagccaatttaactgaactagatatctacagcaggaggctcagccaagaaacaggcctggagatctcagaagaaataaatgaggaggatttgaaggaatgcttctttgatgatatggagagcatcccagctgtcacaacctggaacacctacctgagatacatcacagtgcacaaatccctcatctttgtacttatatggtgccttgtcatcttcttagctgaggtggctgcttccctggtggtgctgtggctgctgggaaacacacccctccaggataaagggaactctactcacagcaggaacaacagttatgctgtgatcatcaccagtacctcctcctactatgtgttctacatttatgttggagttgcagacacattgcttgccatgggtttttttagaggactccccctggtgcatactctcatcactgtttccaaaatccttcaccacaagatgctgcacagtgtactacaggctcccatgagcaccctcaacactcttaaagcaggaggaatcttgaacagatttagcaaggacattgcaattcttgatgacctgcttccactgaccatctttgacttcatccagcttctgctcattgtaattggtgccattgctgtggtagcagtgctccagccatatatttttgtggccactgtgcctgttattgtggccttcattatgttgagagcctacttcctgcagacctctcagcagctcaagcaacttgaaagtgagggcaggagccccatatttacacacttggtcacttccctcaaaggcctctggacactcagagcttttggaagacaaccttattttgaaactctcttccacaaggctctgaatctccacacagccaactggtttctgtatctttcaacactgcgctggttccagatgaggattgagatgatctttgttatcttcttcatagctgttaccttcatctctattctgacaactggtgagggggaagggagagtaggcatcatcctcacactagccatgaacataatgtctaccttacaatgggccgtgaacagctccatagatgtggacagcctcatgagaagtgtgtcaagagttttcaaattcattgacatgcccacagaaggcaaaccaaccaagagcacaaaaccctacaagaatggccagctgagtaaggtcatgatcattgaaaattctcatgtgaagaaggatgatatttggcccagtgggggccagatgacagtcaaggacctcactgccaaatacacagagggtggaaatgctatcctagagaacatctccttctccatctccccaggccaaagagttggcttgctgggcaggactggcagtggcaagtccaccttgctctcagcatttctcaggcttttaaatacagagggagagattcaaattgatggggtgtcttgggatagtataacacttcaacagtggaggaaagcctttggtgtgattcctcagaaagtgtttatcttctctggcactttcagaaaaaatctggacccctatgaacagtggagtgaccaggaaatctggaaggtggcagatgaagtgggcctaagatcagtcatagagcagtttcctggaaagttggattttgtgcttgtagatggaggctgtgtgctgtcccatggccataaacagctaatgtgcctggctaggtcagtgctgagcaaggccaagatcctgctgttagatgagccttcagcccatctggaccctgtgacataccagattatcagaagaactctgaagcaggcctttgctgactgcactgtcatcctgtgtgagcacagaattgaggccatgctggagtgccagcagttccttgttatagaagagaataaggttaggcagtatgacagcattcagaaactgctaaatgaaagatctctcttcaggcaagctatttcaccatctgatagagtgaaactttttccccacagaaattcctctaaatgtaaatctaagccccagatagctgccttgaaagaggagactgaagaagaagtccaggacaccagactgtga

SEQ ID NO: 21 - DNA, 4443 bp, Artificial Sequence
  Synthetic polynucleotide
atgcagagatccccgctggagaaggcatctgtggtgtcaaaactgttctttagctggacaaggcccatccttaggaaagggtacagacagaggttggagctgtcagacatatatcagatcccttcagtggactctgcagacaacctctctgaaaagctggagagggaatgggacagggaactggccagcaaaaaaaaccctaaactgattaatgccctgaggaggtgcttcttttggagattcatgttctatgggatcttcctttacctgggggaggtgactaaagctgttcagcctcttcttctggggaggattattgcctcctatgacccagacaacaaagaagaaagaagcatagccatttacttaggcataggcctctgcttgctcttcatagttagaaccctcctactccacccagccatctttggtctccaccacataggtatgcagatgagaatagcaatgttctccttgatctacaagaagaccctcaagctgtccagcagggtgctggacaagatctccataggccagttagtcagtctactgtccaataacttaaataagtttgatgagggactggcactggcacattttgtgtggattgcccccctccaagtggcccttcttatgggccttatctgggagctgttgcaggcctctgctttctgtggcctgggtttcctcatagtcctagccttattccaggctggactgggcagaatgatgatgaagtatagggaccaaagagcagggaagatttctgaaaggctggttataacttctgagatgattgagaacattcagtcagtgaaagcttactgctgggaagaagctatggaaaaaatgattgaaaatctcagacagactgaattaaagttgaccaggaaagctgcttatgtcagatacttcaactcctcagccttctttttttctggcttctttgttgtattcctttcagtcctcccctatgccctgattaagggcattatcttgaggaaaattttcacaaccatctccttttgtattgtcctcaggatggctgttacaaggcaatttccttgggctgtgcaaacttggtatgatagccttggagcaatcaacaagatccaggatttcctgcaaaagcaggagtacaagacattggaatacaaccttaccaccactgaggtggtgatggaaaatgtgactgccttctgggaggaggggtttggagagctgtttgagaaagccaaacagaacaacaacaatagaaagacctctaatggtgatgattccctgttcttttctaactttagtcttctggggaccccagttctgaaagatattaactttaaaattgaaaggggacagttgctggctgtggctgggtccactggggctgggaagacaagcctgctcatggtgatcatgggagagctggaacccagtgaaggaaagatcaaacactcaggcaggatctccttctgcagccagttctcatggattatgccaggcactattaaagaaaatatcatctttggtgtaagctatgatgagtacaggtatagatctgtaattaaagcctgccagctggaggaagacatctctaagtttgctgagaaggataacattgtgttgggggaagggggcatcaccctttctggtgggcagagggctaggatctcccttgctagggcagtatacaaggatgctgacttgtacctcttggatagtccttttggctacctagatgtgctgacagagaaagaaatatttgaaagctgtgtgtgtaagctcatggctaacaagaccaggatcctggtcaccagtaaaatggaacacctcaaaaaagcagacaagatccttattctccatgagggctcctcctacttctatgggaccttcagtgagctgcagaatctgcagccagacttctcctcaaaacttatgggctgtgactcctttgaccaattctctgcagaaagaaggaatagcatactgacagaaacactgcatagattctccctggaaggagatgccccagtgagttggacagaaaccaaaaagcagagcttcaagcagactggtgagtttggtgaaaagaggaagaattctatcctgaaccccatcaatagcatcaggaaatttagcatagtccaaaagacccccctccagatgaatggaatagaggaggatagtgatgagcctcttgagagaaggctgtccctggttccagacagtgaacagggtgaagccattcttccgaggatcagtgtcatctccactgggcccacattgcaggccagaagaagacagtctgttctgaatttgatgacacattctgtgaatcaaggccagaatatccatagaaaaaccactgccagcaccagaaaagtttctctagccccccaggctaacctgactgagttagacatctacagcagaaggctgagccaagagactggcttggaaatatctgaggagatcaatgaggaggacctcaaggagtgcttctttgatgacatggagtcaatccctgcagtcactacatggaacacttacctaaggtacatcacagttcataagagcctcatctttgtcctcatatggtgtctggtcatctttttagcagaagtggctgccagcctagttgtgctgtggttactgggcaatacacctcttcaggacaaaggcaatagcacacacagcagaaacaactcctatgcagtgatcatcacctctacaagctcttactatgtattctatatatatgtgggagtggcagatactctcctggccatgggattcttcaggggattacctctagttcacacattgatcacagtgtcaaaaattctccaccacaagatgttacacagtgtcctgcaagccccaatgtctactctgaacacacttaaggcaggtggaattttgaataggtttagcaaggacatagctatcctggatgatctcctccctctgaccatctttgacttcatccagttactgctcattgtaattggagccattgcagtggtagcagtcctacagccttacatttttgtggctactgttcctgttattgtggccttcattatgctaagagcttacttcctgcaaacaagccaacagttgaaacagctagaaagtgagggaaggtcccccatcttcacccacctggtgacatcactcaaggggctatggactcttagggcttttgggagacagccgtactttgagaccttattccataaggcccttaacctccatacagcaaactggttcttatacctgagtactctgaggtggtttcaaatgaggattgaaatgatttttgtgatcttcttcattgctgtgaccttcatctcaatcttgaccacaggagagggggagggcagggtgggcatcatactgaccttggccatgaacattatgtcaaccctgcagtgggctgtcaatagctccattgatgtggacagtctgatgaggagtgtctccagggtcttcaagtttattgacatgccaactgagggcaaacccaccaaaagcactaagccatataaaaatggccaactgtccaaagtgatgatcattgaaaattcacatgtaaagaaggatgatatctggccctctggaggacagatgacagtgaaagacctgactgccaagtacacagagggtggtaatgccattcttgagaacattagtttcagtatttccccggggcaaagggtgggcctccttggcagaacaggctctggcaagagtaccctgctgtcagcctttttaagactgttgaacactgagggagaaattcagattgatggtgtctcctgggatagcatcaccctccagcagtggagaaaagcttttggagtgatcccgcaaaaggttttcatcttttcaggcaccttccggaagaacctggacccctatgagcagtggtctgaccaggaaatatggaaggtagctgatgaagttgggcttaggtcagtcatagagcagttcccaggcaaactggactttgtcctggtggatggtggatgtgtactgagtcatgggcacaaacagctgatgtgcctagccaggtctgtgctcagcaaggcaaagatattgctgcttgatgaacccagtgcccatctggacccagtcacatatcagatcatcagaagaacattgaagcaggcctttgctgattgcacagttatcctctgtgagcacaggattgaggccatgctggagtgccagcagtttctggtgattgaggagaataaagtaaggcagtatgactccatccagaagctgctcaatgaaagaagcctctttagacaagctatctccccctcagacagggtcaaattgttccctcacagaaacagcagcaagtgcaagagcaagccccaaattgcagccttgaaagaggagacagaggaagaggtgcaggacaccagactctga

SEQ ID NO: 22 - DNA, 4443 bp, Artificial Sequence
  Synthetic polynucleotide
atgcagagaagccccctggagaaggccagcgtggtgagcaagctgttcttcagctggaccagacccatcctgagaaagggctacagacagagactggagctgagcgacatctaccagatccccagcgtggacagcgccgacaacctgagcgagaagctggagagagagtgggacagagagctggccagcaagaagaaccccaagctgatcaacgccctgagaagatgcttcttctggagattcatgttctacggcatcttcctgtacctgggcgaggtgaccaaggccgtgcagcccctgctgctgggcagaatcatcgccagctacgaccccgacaacaaggaggagagaagcatcgccatctacctgggcatcggcctgtgcctgctgttcatcgtgagaaccctgctgctgcaccccgccatcttcggcctgcaccacatcggcatgcagatgagaatcgccatgttcagcctgatctacaagaagaccctgaagctgagcagcagagtgctggacaagatcagcatcggccagctggtgagcctgctgagcaacaacctgaacaagttcgacgagggcctggccctggcccacttcgtgtggatcgcccccctgcaggtggccctgctgatgggcctgatctgggagctgctgcaggccagcgccttctgcggcctgggcttcctgatcgtgctggccctgttccaggccggcctgggcagaatgatgatgaagtacagagaccagagagccggcaagatcagcgagagactggtgatcaccagcgagatgatcgagaacatccagagcgtgaaggcctactgctgggaggaggccatggagaagatgatcgagaacctgagacagaccgagctgaagctgaccagaaaggccgcctacgtgagatacttcaacagcagcgccttcttcttcagcggcttcttcgtggtgttcctgagcgtgctgccctacgccctgatcaagggcatcatcctgagaaagatcttcaccaccatcagcttctgcatcgtgctgagaatggccgtgaccagacagttcccctgggccgtgcagacctggtacgacagcctgggcgccatcaacaagatccaggacttcctgcagaagcaggagtacaagaccctggagtacaacctgaccaccaccgaggtggtgatggagaacgtgaccgccttctgggaggagggcttcggcgagctgttcgagaaggccaagcagaacaacaacaacagaaagaccagcaacggcgacgacagcctgttcttcagcaacttcagcctgctgggcacccccgtgctgaaggacatcaacttcaagatcgagagaggccagctgctggccgtggccggcagcaccggcgccggcaagaccagcctgctgatggtgatcatgggcgagctggagcccagcgagggcaagatcaagcacagcggcagaatcagcttctgcagccagttcagctggatcatgcccggcaccatcaaggagaacatcatcttcggcgtgagctacgacgagtacagatacagaagcgtgatcaaggcctgccagctggaggaggacatcagcaagttcgccgagaaggacaacatcgtgctgggcgagggcggcatcaccctgagcggcggccagagagccagaatcagcctggccagagccgtgtacaaggacgccgacctgtacctgctggacagccccttcggctacctggacgtgctgaccgagaaggagatcttcgagagctgcgtgtgcaagctgatggccaacaagaccagaatcctggtgaccagcaagatggagcacctgaagaaggccgacaagatcctgatcctgcacgagggcagcagctacttctacggcaccttcagcgagctgcagaacctgcagcccgacttcagcagcaagctgatgggctgcgacagcttcgaccagttcagcgccgagagaagaaacagcatcctgaccgagaccctgcacagattcagcctggagggcgacgcccccgtgagctggaccgagaccaagaagcagagcttcaagcagaccggcgagttcggcgagaagagaaagaacagcatcctgaaccccatcaacagcatcagaaagttcagcatcgtgcagaagacccccctgcagatgaacggcatcgaggaggacagcgacgagcccctggagagaagactgagcctggtgcccgacagcgagcagggcgaggccatcctgcccagaatcagcgtgatcagcaccggccccaccctgcaggccagaagaagacagagcgtgctgaacctgatgacccacagcgtgaaccagggccagaacatccacagaaagaccaccgccagcaccagaaaggtgagcctggccccccaggccaacctgaccgagctggacatctacagcagaagactgagccaggagaccggcctggagatcagcgaggagatcaacgaggaggacctgaaggagtgcttcttcgacgacatggagagcatccccgccgtgaccacctggaacacctacctgagatacatcaccgtgcacaagagcctgatcttcgtgctgatctggtgcctggtgatcttcctggccgaggtggccgccagcctggtggtgctgtggctgctgggcaacacccccctgcaggacaagggcaacagcacccacagcagaaacaacagctacgccgtgatcatcaccagcaccagcagctactacgtgttctacatctacgtgggcgtggccgacaccctgctggccatgggcttcttcagaggcctgcccctggtgcacaccctgatcaccgtgagcaagatcctgcaccacaagatgctgcacagcgtgctgcaggcccccatgagcaccctgaacaccctgaaggccggcggcatcctgaacagattcagcaaggacatcgccatcctggacgacctgctgcccctgaccatcttcgacttcatccagctgctgctgatcgtgatcggcgccatcgccgtggtggccgtgctgcagccctacatcttcgtggccaccgtgcccgtgatcgtggccttcatcatgctgagagcctacttcctgcagaccagccagcagctgaagcagctggagagcgagggcagaagccccatcttcacccacctggtgaccagcctgaagggcctgtggaccctgagagccttcggcagacagccctacttcgagaccctgttccacaaggccctgaacctgcacaccgccaactggttcctgtacctgagcaccctgagatggttccagatgagaatcgagatgatcttcgtgatcttcttcatcgccgtgaccttcatcagcatcctgaccaccggcgagggcgagggcagagtgggcatcatcctgaccctggccatgaacatcatgagcaccctgcagtgggccgtgaacagcagcatcgacgtggacagcctgatgagaagcgtgagcagagtgttcaagttcatcgacatgcccaccgagggcaagcccaccaagagcaccaagccctacaagaacggccagctgagcaaggtgatgatcatcgagaacagccacgtgaagaaggacgacatctggcccagcggcggccagatgaccgtgaaggacctgaccgccaagtacaccgagggcggcaacgccatcctggagaacatcagcttcagcatcagccccggccagagagtgggcctgctgggcagaaccggcagcggcaagagcaccctgctgagcgccttcctgagactgctgaacaccgagggcgagatccagatcgacggcgtgagctgggacagcatcaccctgcagcagtggagaaaggccttcggcgtgatcccccagaaggtgttcatcttcagcggcaccttcagaaagaacctggacccctacgagcagtggagcgaccaggagatctggaaggtggccgacgaggtgggcctgagaagcgtgatcgagcagttccccggcaagctggacttcgtgctggtggacggcggctgcgtgctgagccacggccacaagcagctgatgtgcctggccagaagcgtgctgagcaaggccaagatcctgctgctggacgagcccagcgcccacctggaccccgtgacctaccagatcatcagaagaaccctgaagcaggccttcgccgactgcaccgtgatcctgtgcgagcacagaatcgaggccatgctggagtgccagcagttcctggtgatcgaggagaacaaggtgagacagtacgacagcatccagaagctgctgaacgagagaagcctgttcagacaggccatcagccccagcgacagagtgaagctgttcccccacagaaacagcagcaagtgcaagagcaagccccagatcgccgccctgaaggaggagaccgaggaggaggtgcaggacaccagactgtga

SEQ ID NO: 23 - DNA, 4443 bp, Artificial Sequence
  Synthetic polynucleotide
atgcagcgcagccccctggagaaggccagcgtggtgagcaagctgttcttcagctggacccgccccatcctgcgcaagggctaccgccagcgcctggagctgagcgacatctaccagatccccagcgtggacagcgccgacaacctgagcgagaagctggagcgcgagtgggaccgcgagctggccagcaagaagaaccccaagctgatcaacgccctgcgccgctgcttcttctggcgcttcatgttctacggcatcttcctgtacctgggcgaggtgaccaaggccgtgcagcccctgctgctgggccgcatcatcgccagctacgaccccgacaacaaggaggagcgcagcatcgccatctacctgggcatcggcctgtgcctgctgttcatcgtgcgcaccctgctgctgcaccccgccatcttcggcctgcaccacatcggcatgcagatgcgcatcgccatgttcagcctgatctacaagaagaccctgaagctgagcagccgcgtgctggacaagatcagcatcggccagctggtgagcctgctgagcaacaacctgaacaagttcgacgagggcctggccctggcccacttcgtgtggatcgcccccctgcaggtggccctgctgatgggcctgatctgggagctgctgcaggccagcgccttctgcggcctgggcttcctgatcgtgctggccctgttccaggccggcctgggccgcatgatgatgaagtaccgcgaccagcgcgccggcaagatcagcgagcgcctggtgatcaccagcgagatgatcgagaacatccagagcgtgaaggcctactgctgggaggaggccatggagaagatgatcgagaacctgcgccagaccgagctgaagctgacccgcaaggccgcctacgtgcgctacttcaacagcagcgccttcttcttcagcggcttcttcgtggtgttcctgagcgtgctgccctacgccctgatcaagggcatcatcctgcgcaagatcttcaccaccatcagcttctgcatcgtgctgcgcatggccgtgacccgccagttcccctgggccgtgcagacctggtacgacagcctgggcgccatcaacaagatccaggacttcctgcagaagcaggagtacaagaccctggagtacaacctgaccaccaccgaggtggtgatggagaacgtgaccgccttctgggaggagggcttcggcgagctgttcgagaaggccaagcagaacaacaacaaccgcaagaccagcaacggcgacgacagcctgttcttcagcaacttcagcctgctgggcacccccgtgctgaaggacatcaacttcaagatcgagcgcggccagctgctggccgtggccggcagcaccggcgccggcaagaccagcctgctgatggtgatcatgggcgagctggagcccagcgagggcaagatcaagcacagcggccgcatcagcttctgcagccagttcagctggatcatgcccggcaccatcaaggagaacatcatcttcggcgtgagctacgacgagtaccgctaccgcagcgtgatcaaggcctgccagctggaggaggacatcagcaagttcgccgagaaggacaacatcgtgctgggcgagggcggcatcaccctgagcggcggccagcgcgcccgcatcagcctggcccgcgccgtgtacaaggacgccgacctgtacctgctggacagccccttcggctacctggacgtgctgaccgagaaggagatcttcgagagctgcgtgtgcaagctgatggccaacaagacccgcatcctggtgaccagcaagatggagcacctgaagaaggccgacaagatcctgatcctgcacgagggcagcagctacttctacggcaccttcagcgagctgcagaacctgcagcccgacttcagcagcaagctgatgggctgcgacagcttcgaccagttcagcgccgagcgccgcaacagcatcctgaccgagaccctgcaccgcttcagcctggagggcgacgcccccgtgagctggaccgagaccaagaagcagagcttcaagcagaccggcgagttcggcgagaagcgcaagaacagcatcctgaaccccatcaacagcatccgcaagttcagcatcgtgcagaagacccccctgcagatgaacggcatcgaggaggacagcgacgagcccctggagcgccgcctgagcctggtgcccgacagcgagcagggcgaggccatcctgccccgcatcagcgtgatcagcaccggccccaccctgcaggcccgccgccgccagagcgtgctgaacctgatgacccacagcgtgaaccagggccagaacatccaccgcaagaccaccgccagcacccgcaaggtgagcctggccccccaggccaacctgaccgagctggacatctacagccgccgcctgagccaggagaccggcctggagatcagcgaggagatcaacgaggaggacctgaaggagtgcttcttcgacgacatggagagcatccccgccgtgaccacctggaacacctacctgcgctacatcaccgtgcacaagagcctgatcttcgtgctgatctggtgcctggtgatcttcctggccgaggtggccgccagcctggtggtgctgtggctgctgggcaacacccccctgcaggacaagggcaacagcacccacagccgcaacaacagctacgccgtgatcatcaccagcaccagcagctactacgtgttctacatctacgtgggcgtggccgacaccctgctggccatgggcttcttccgcggcctgcccctggtgcacaccctgatcaccgtgagcaagatcctgcaccacaagatgctgcacagcgtgctgcaggcccccatgagcaccctgaacaccctgaaggccggcggcatcctgaaccgcttcagcaaggacatcgccatcctggacgacctgctgcccctgaccatcttcgacttcatccagctgctgctgatcgtgatcggcgccatcgccgtggtggccgtgctgcagccctacatcttcgtggccaccgtgcccgtgatcgtggccttcatcatgctgcgcgcctacttcctgcagaccagccagcagctgaagcagctggagagcgagggccgcagccccatcttcacccacctggtgaccagcctgaagggcctgtggaccctgcgcgccttcggccgccagccctacttcgagaccctgttccacaaggccctgaacctgcacaccgccaactggttcctgtacctgagcaccctgcgctggttccagatgcgcatcgagatgatcttcgtgatcttcttcatcgccgtgaccttcatcagcatcctgaccaccggcgagggcgagggccgcgtgggcatcatcctgaccctggccatgaacatcatgagcaccctgcagtgggccgtgaacagcagcatcgacgtggacagcctgatgcgcagcgtgagccgcgtgttcaagttcatcgacatgcccaccgagggcaagcccaccaagagcaccaagccctacaagaacggccagctgagcaaggtgatgatcatcgagaacagccacgtgaagaaggacgacatctggcccagcggcggccagatgaccgtgaaggacctgaccgccaagtacaccgagggcggcaacgccatcctggagaacatcagcttcagcatcagccccggccagcgcgtgggcctgctgggccgcaccggcagcggcaagagcaccctgctgagcgccttcctgcgcctgctgaacaccgagggcgagatccagatcgacggcgtgagctgggacagcatcaccctgcagcagtggcgcaaggccttcggcgtgatcccccagaaggtgttcatcttcagcggcaccttccgcaagaacctggacccctacgagcagtggagcgaccaggagatctggaaggtggccgacgaggtgggcctgcgcagcgtgatcgagcagttccccggcaagctggacttcgtgctggtggacggcggctgcgtgctgagccacggccacaagcagctgatgtgcctggcccgcagcgtgctgagcaaggccaagatcctgctgctggacgagcccagcgcccacctggaccccgtgacctaccagatcatccgccgcaccctgaagcaggccttcgccgactgcaccgtgatcctgtgcgagcaccgcatcgaggccatgctggagtgccagcagttcctggtgatcgaggagaacaaggtgcgccagtacgacagcatccagaagctgctgaacgagcgcagcctgttccgccaggccatcagccccagcgaccgcgtgaagctgttcccccaccgcaacagcagcaagtgcaagagcaagccccagatcgccgccctgaaggaggagaccgaggaggaggtgcaggacacccgcctgtaa

SEQ ID NO: 24 - DNA, 4443 bp, Artificial Sequence
  Synthetic polynucleotide
atgcagagaagccccctggagaaggccagcgtggtgagcaagctgttcttcagctggaccagacccatcctgagaaagggctacagacagagactggagctgagcgacatctaccagatccccagcgtggacagcgccgacaacctgagcgagaagctggagagagagtgggacagagagctggccagcaagaagaaccccaagctgatcaacgccctgagaagatgcttcttctggagattcatgttctacggcatcttcctgtacctgggcgaggtgaccaaggccgtgcagcccctgctgctgggcagaatcatcgccagctacgaccccgacaacaaggaggagagaagcatcgccatctacctgggcatcggcctgtgcctgctgttcatcgtgagaaccctgctgctgcaccccgccatcttcggcctgcaccacatcggcatgcagatgagaatcgccatgttcagcctgatctacaagaagaccctgaagctgagcagcagagtgctggacaagatcagcatcggccagctggtgagcctgctgagcaacaacctgaacaagttcgacgagggcctggccctggcccacttcgtgtggatcgcccccctgcaggtggccctgctgatgggcctgatctgggagctgctgcaggccagcgccttctgcggcctgggcttcctgatcgtgctggccctgttccaggccggcctgggcagaatgatgatgaagtacagggaccagagagccggcaagatcagcgagagactggtgatcaccagcgagatgatcgagaacatccagagcgtgaaggcctactgctgggaggaggccatggagaagatgatcgagaacctgagacagaccgagctgaagctgaccagaaaggccgcctacgtgagatacttcaacagcagcgccttcttcttcagcggcttcttcgtggtgttcctgagcgtgctgccctacgccctgatcaagggcatcatcctgagaaagatcttcaccaccatcagcttctgcatcgtgctgagaatggccgtgaccagacagttcccctgggccgtgcagacctggtacgacagcctgggcgccatcaacaagatccaggacttcctgcagaagcaggagtacaagaccctggagtacaacctgaccaccaccgaggtggtgatggagaacgtgaccgccttctgggaggagggcttcggcgagctgttcgagaaggccaagcagaacaacaacaacagaaagaccagcaacggcgacgacagcctgttcttcagcaacttcagcctgctgggcacccccgtgctgaaggacatcaacttcaagatcgagagaggccagctgctggccgtggccggcagcaccggcgccggcaagaccagcctgctgatggtgatcatgggcgagctggagcccagcgagggcaagatcaagcacagcggcagaatcagcttctgcagccagttcagctggatcatgcccggcaccatcaaggagaacatcatcttcggcgtgagctacgacgagtacagatacagaagcgtgatcaaggcctgccagctggaggaggacatcagcaagttcgccgagaaggacaacatcgtgctgggcgagggcggcatcaccctgagcggcggccagagagccagaatcagcctggccagagccgtgtacaaggacgccgacctgtacctgctggacagccccttcggctacctggacgtgctgaccgagaaggagatcttcgagagctgcgtgtgcaagctgatggccaacaagaccagaatcctggtgaccagcaagatggagcacctgaagaaggccgacaagatcctgatcctgcacgagggcagcagctacttctacggcaccttcagcgagctgcagaacctgcagcccgacttcagcagcaagctgatgggctgcgacagcttcgaccagttcagcgccgagagaagaaacagcatcctgaccgagaccctgcacagattcagcctggagggcgacgcccccgtgagctggaccgagaccaagaagcagagcttcaagcagaccggcgagttcggcgagaagagaaagaacagcatcctgaaccccatcaacagcatcagaaagttcagcatcgtgcagaagacccccctgcagatgaacggcatcgaggaggacagcgacgagcccctggagagaagactgagcctggtgcccgacagcgagcagggcgaggccatcctgcccagaatcagcgtgatcagcaccggccccaccctgcaggccagaagaagacagagcgtgctgaacctgatgacccacagcgtgaaccagggccagaacatccacagaaagaccaccgccagcaccagaaaggtgagcctggccccccaggccaacctgaccgagctggacatctacagcagaagactgagccaggagaccggcctggagatcagcgaggagatcaacgaggaggacctgaaggagtgcttcttcgacgacatggagagcatccccgccgtgaccacctggaacacctacctgagatacatcaccgtgcacaagagcctgatcttcgtgctgatctggtgcctggtgatcttcctggccgaggtggccgccagcctggtggtgctgtggctgctgggcaacacccccctgcaggacaagggcaacagcacccacagcagaaacaacagctacgccgtgatcatcaccagcaccagcagctactacgtgttctacatctacgtgggcgtggccgacaccctgctggccatgggcttcttcagaggcctgcccctggtgcacaccctgatcaccgtgagcaagatcctgcaccacaagatgctgcacagcgtgctgcaggcccccatgagcaccctgaacaccctgaaggccggcggcatcctgaacagattcagcaaggacatcgccatcctggacgacctgctgcccctgaccatcttcgacttcatccagctgctgctgatcgtgatcggcgccatcgccgtggtggccgtgctgcagccctacatcttcgtggccaccgtgcccgtgatcgtggccttcatcatgctgagagcctacttcctgcagaccagccagcagctgaagcagctggagagcgagggcaggagccccatcttcacccacctggtgaccagcctgaagggcctgtggaccctgagagccttcggcagacagccctacttcgagaccctgttccacaaggccctgaacctgcacaccgccaactggttcctgtacctgagcaccctgagatggttccagatgagaatcgagatgatcttcgtgatcttcttcatcgccgtgaccttcatcagcatcctgaccaccggcgagggcgagggcagagtgggcatcatcctgaccctggccatgaacatcatgagcaccctgcagtgggccgtgaacagcagcatcgacgtggacagcctgatgagaagcgtgagcagagtgttcaagttcatcgacatgcccaccgagggcaagcccaccaagagcaccaagccctacaagaacggccagctgagcaaggtgatgatcatcgagaacagccacgtgaagaaggacgacatctggcccagcggcggccagatgaccgtgaaggacctgaccgccaagtacaccgagggcggcaacgccatcctggagaacatcagcttcagcatcagccccggccagagagtgggcctgctgggcagaaccggcagcggcaagagcaccctgctgagcgccttcctgagactgctgaacaccgagggcgagatccagatcgacggcgtgagctgggacagcatcaccctgcagcagtggagaaaggccttcggcgtgatcccccagaaggtgttcatcttcagcggcaccttcagaaagaacctggacccctacgagcagtggagcgaccaggagatctggaaggtggccgacgaggtgggcctgagaagcgtgatcgagcagttccccggcaagctggacttcgtgctggtggacggcggctgcgtgctgagccacggccacaagcagctgatgtgcctggccagaagcgtgctgagcaaggccaagatcctgctgctggacgagcccagcgcccacctggaccccgtgacctaccagatcatcagaagaaccctgaagcaggccttcgccgactgcaccgtgatcctgtgcgagcacagaatcgaggccatgctggagtgccagcagttcctggtgatcgaggagaacaaggtgagacagtacgacagcatccagaagctgctgaacgagagaagcctgttcagacaggccatcagccccagcgacagagtgaagctgttcccccacagaaacagcagcaagtgcaagagcaagccccagatcgccgccctgaaggaggagaccgaggaggaggtgcaggacaccagactgtga

SEQ ID NO: 25 - DNA, 4443 bp, Artificial Sequence
  Synthetic polynucleotide
atgcagaggtcacctctggaaaaggctagcgtggtcagcaagctatttttttcctggacccgcccgatactcaggaagggctaccgacagcggctggagctgagtgacatttatcagattccctccgtcgattccgctgacaacctgtctgagaaactggagcgggaatgggatagggaactggcgtccaaaaaaaaccccaaactcatcaatgcactccgcagatgcttcttctggcggtttatgttttatggcatattcctgtatctgggggaggtgacgaaagccgtgcagccgctgctgcttggtcgcattatcgcgtcatacgatccagataacaaggaggaaagaagtatcgctatctatctcgggatagggctgtgcctgctcttcattgtgcggactcttctcttgcaccccgccattttcggtctgcatcatataggtatgcagatgagaattgcgatgttctcattgatttacaaaaaaacgcttaagctaagttcaagggtgctagataagatatcgatcggccagctggtgtctctgcttagcaacaacctcaataaattcgacgaaggccttgcactggcccacttcgtgtggatcgcccctctgcaggtggctctgctgatggggttaatatgggagctgttgcaggcctccgctttttgtggcctggggtttctcatcgtgttggccttgtttcaggcagggctgggacgtatgatgatgaaatatagggatcagagggctggcaaaatctctgagcgcctggttattacgagtgaaatgattgagaacatccagtcagtgaaggcctattgctgggaggaggccatggaaaaaatgattgagaacctacgccagactgagctgaagttaaccagaaaagccgcctatgtgcgctactttaacagtagcgcatttttcttctccggttttttcgtggtgtttcttagtgtgttgccgtatgccttaatcaagggaataatactccggaagattttcactaccatcagcttctgtatcgtgttgcggatggccgtcacccggcagtttccctgggcagtacagacttggtacgattctctcggagcaattaacaaaatccaagactttctacaaaagcaggagtacaagaccctggagtacaatctgaccaccacagaagtcgtaatggagaatgtaactgccttctgggaagagggctttggcgaactctttgaaaaggccaagcagaacaataacaaccggaagacctccaacggggacgacagcttatttttcagcaatttttctttgctcgggacccctgtactgaaagatattaactttaagatcgagcgcggacaactcctggctgtcgccggcagcactggagctggaaaaacatcactgcttatggtgataatgggagaactcgaaccaagcgagggaaaaataaagcactctggacggattagtttttgctcccagttctcgtggataatgcctggcaccattaaggagaatatcatctttggagtgagttacgacgaataccggtaccggtccgttatcaaggcttgtcaactcgaggaggacatttctaaattcgccgaaaaagataatatagtgctgggcgaaggaggcattacactgagcgggggtcagagagctcgaattagcctcgcccgagcagtctataaagacgccgatctttacctgctggattccccttttgggtatttggatgttctgacagagaaggaaatctttgaatcatgtgtctgtaaactgatggccaataagactaggattctagtgacttcgaaaatggagcacctgaaaaaagcggacaaaattctgatactccatgaagggtcttcctacttctacggcaccttctcagagttgcagaacttacaacctgatttttcatctaagcttatggggtgcgactcgtttgaccagttctccgctgaaagacgaaacagcatcttaacggaaactcttcacaggttctcattagagggagatgcgccggtgtcctggacagagacaaaaaaacagtctttcaaacagacaggagagtttggcgagaagagaaaaaactcaatcctcaatcccatcaattctattagaaagtttagcatcgtccaaaaaacaccattgcagatgaatgggattgaggaggacagtgatgagcctttggaacgaagactgtccctggtacccgatagcgaacagggtgaggccatccttcctaggatctcggtcataagtacagggcccacactgcaggccaggcgacgtcaaagtgtcctcaatcttatgacgcacagtgtgaatcaggggcagaacatccatcgtaagacgacagcttcaactcgaaaggtcagtctagctccacaagccaatcttacagagctggacatttattcccgccgcctcagtcaggagaccggattggaaatatcagaggaaattaatgaagaggatctgaaggaatgcttctttgatgacatggaatcgatccccgctgttactacctggaacacatatctgagatatattaccgtccataagagcttaatctttgtactgatatggtgcttggtgattttcctggcagaggttgcggcgagtttggtcgtgctatggctccttggaaacactcccctgcaggataaggggaactccactcatagcaggaataacagctatgccgtgatcatcacctctacctcctcttattacgtgttttacatatacgtcggtgttgcggataccctgttggcaatggggttctttagaggactacccctagttcacaccctgatcaccgtttcgaagatcttgcaccacaagatgcttcatagcgttctccaagctcctatgagcacccttaatacactgaaagcaggaggtatccttaaccgcttttccaaagacatcgctatactcgacgatttgctcccattgaccatcttcgacttcattcagctgctcctcattgtgatcggcgccattgccgtggtcgcagtgttacagccatatattttcgtagccaccgtgcccgtcatcgtggcatttatcatgctgcgcgcatatttcttacagacatctcagcaactgaagcagctggaatctgagggcagatctcctatttttacacacctggttaccagcctgaagggcctgtggaccctgcgtgctttcggtcgccaaccctactttgagactctcttccataaggctctgaatttacatactgccaattggttcctataccttagtacccttcggtggttccagatgcggatagaaatgatcttcgtgattttcttcatcgcagtcactttcatctctattttgacgaccggtgagggcgagggcagggtgggcatcattctgactttggccatgaacattatgtcaacactccagtgggccgttaattcaagcattgatgtggattccttgatgcgttccgtcagcagggtatttaaattcatagacatgcccaccgagggcaagccaacaaaatctaccaagccatacaaaaatggccaactaagcaaggtcatgattatcgagaattctcatgtgaaaaaggacgacatttggccttccgggggtcaaatgactgtaaaggacctgacggctaaatacactgagggcggtaatgctatcttggagaacatctctttcagcatctcccctggccagagagtgggactgctcgggcggacaggctccggaaagtctacgctcctttcagcattccttagacttctgaacaccgaaggtgagattcagattgacggggtctcttgggactccatcacacttcagcaatggaggaaggcattcggtgtaatcccccaaaaggtttttatcttctccggaacatttcgtaagaatctggacccgtacgagcagtggtcagatcaggagatctggaaagtagcagacgaggtcgggctacggagcgttattgaacagtttcctggcaaactggacttcgttttggtggacggaggctgtgtgctgagtcacggccataaacaactgatgtgcttagctaggtctgttctcagcaaggcaaagattttactgctggatgaaccaagcgcccaccttgatccagtgacatatcaaatcatcagaagaactcttaaacaggcgttcgccgactgcacagtgatcctgtgtgagcacagaatagaagccatgctggaatgtcaacagtttctcgtgattgaggagaacaaggtgcgccagtacgatagcatccagaagttactcaatgaaaggtcactcttcaggcaggccatctcacccagcgaccgcgttaagctgtttccacaccgaaacagttccaagtgcaaaagtaagccacagattgctgcactgaaggaagagacagaagaagaagttcaggacactcggctctga

SEQ ID NO: 26 - DNA, 4443 bp, Artificial Sequence; identical to SEQ ID NO: 8
  Synthetic polynucleotide

SEQ ID NO: 27 - DNA, 4443 bp, Artificial Sequence
  Synthetic polynucleotide
atgcaacggagtcctctggaaaaagcctctgtcgtatctaagcttttcttcagttggacacgcccgattttgagaaagggttatcggcaacgcttggaacttagtgacatctaccaaattccaagtgtagactcagccgataacttgagcgaaaagctcgaacgagagtgggatcgagaactggctagcaaaaaaaatcccaaactcataaatgccctgcgacgctgtttcttttggcgatttatgttttacggtattttcctttatttgggtgaggtcacgaaggctgtacagccactgctgctgggtcgcatcattgcctcttacgaccctgacaacaaagaggagcggtcaatagctatctaccttggtataggactttgcttgctcttcatagtccgcacgttgcttctccaccctgctatatttggtctccatcacattgggatgcaaatgcggatcgcgatgttcagtcttatatataaaaagactcttaaactttccagccgggttctggataagatctctattggtcaactggtatctcttttgtctaacaacctgaataagttcgacgagggccttgcattggcccattttgtatggattgcccctttgcaagtcgccctcctgatgggattgatctgggaactcctgcaagctagtgctttttgcggattgggattcctcatagtccttgcgctctttcaggcgggacttggacgcatgatgatgaagtatcgcgaccaacgagctggcaagatcagtgaacggcttgtaataaccagtgaaatgatagagaacatccagagcgtaaaagcttactgttgggaagaagcgatggaaaagatgattgagaaccttcgccagacagaacttaaacttacacgaaaggccgcttatgtccggtacttcaactcttcagcatttttttttagtggcttctttgtagtgttcctgtccgtccttccgtatgcacttatcaagggtataatacttaggaaaatcttcacaacaatcagtttttgcatagtccttcgcatggcagtaactcgccaatttccctgggcagttcagacgtggtacgactcacttggcgcaattaacaaaattcaagatttcctccaaaagcaagagtataaaaccttggaatacaaccttaccaccacagaagttgtaatggaaaatgtcacagccttctgggaggaaggtttcggcgaactttttgagaaggcgaagcaaaataacaataatcggaaaacatcaaacggtgacgattcactgttcttttctaactttagccttcttgggacgcccgtcctgaaggacataaactttaagattgaacggggtcaacttctcgcggtcgcagggagtactggagcggggaaaacgagcctgctgatggtgataatgggggagttggagccctcagaaggcaagatcaagcatagtggtagaattagcttctgcagtcaatttagttggattatgccgggcacgatcaaagaaaatataatctttggggtatcctacgatgaatacaggtaccgatcagtgataaaagcgtgccagcttgaagaagacatttcaaagtttgctgagaaggataatatcgtacttggagaaggaggtatcaccctgtctgggggtcaacgagcgaggatctccctggcacgcgccgtctacaaggacgcggacctctatctgttggattcaccgttcggatatttggacgtgcttacggagaaagaaatatttgagagctgtgtttgcaagctcatggcaaataaaaccagaatattggttacaagcaagatggagcatcttaagaaagcagataaaatcctgatattgcacgagggctcttcatacttctacgggacgttttctgagttgcagaacctccagccggatttcagctctaagctgatgggctgtgattcctttgatcagtttagtgcggaaagacgaaacagtatactcaccgaaacactgcacaggttctctctggagggcgacgccccggtttcctggacagagacgaagaagcagtccttcaaacagacaggcgagtttggggagaaaaggaaaaatagcatactcaacccgattaacagcattcgcaagttcagtatagtacaaaagaccccgttgcagatgaacggtatagaggaagattctgatgagccactggaaagacggctttctctcgttccggacagtgaacagggagaggcaatactgcctcggatcagcgttatctctacaggacctactttgcaagctcggcgccgacagtcagtcttgaatcttatgactcatagtgttaatcaaggccagaatatccatcgcaagaccaccgcaagtacaaggaaagtgagcttggcacctcaagcaaaccttactgaacttgatatctactcacggcgactttcacaggagaccggacttgaaattagtgaagaaattaacgaggaggacctcaaggagtgcttcttcgatgacatggaatcaatccccgcagtcacaacctggaacacttatctgaggtatataacagttcacaagagcctcatttttgtacttatttggtgtttggtaattttcctggcggaggttgctgcttctttggtcgtcctttggctcctcgggaatacaccgctccaagacaaaggcaactctacccatagtaggaacaattcatatgcagtgattataaccagtacatcatcttattacgttttctatatttatgtcggggtagctgacacgctgttggcgatgggcttctttaggggcctccccttggtacacacccttatcacggtgagtaaaatcctgcatcacaaaatgcttcattctgtactccaagcgccgatgagtacgcttaatacgctgaaagcaggagggatactgaatcggttcagcaaggacatcgccattctggatgacctgcttccattgacaatatttgatttcattcagctccttctcatagttattggagccatagcggtggtggctgtgcttcagccttatatattcgttgccacagttcccgttatagtggcatttataatgctcagggcctactttctccagacttcccagcagttgaagcaactcgaatcagaaggaaggtcacctattttcacacatcttgtgacttccttgaagggcttgtggacgctgcgggccttcggaagacaaccatattttgaaactctcttccacaaagctttgaatcttcatactgcgaactggttcctgtatttgagtactttgcgctggttccagatgaggatagaaatgatattcgttatcttctttatcgcggttacgttcataagtatcctcactacgggggagggtgagggtagagtgggcataatactgaccctcgccatgaacattatgtccaccctgcagtgggcggtaaacagcagcatagatgtggattctttgatgcgcagtgtgagcagggtttttaagtttatcgatatgccgacggaaggaaagcccactaaaagcacgaaaccctataaaaatggacagcttagcaaagtaatgataatcgagaatagccatgtgaaaaaggatgacatatggccttccggaggccaaatgactgttaaagatctgaccgctaaatataccgagggcggcaacgcaatactcgaaaacataagcttttccataagccccggccaacgcgtgggtcttctggggaggactggctccggaaaatcaacgttgcttagcgcgtttttgcggctccttaacactgaaggtgagatccaaatagatggcgttagttgggactctataacactgcaacaatggcggaaagctttcggcgtcatacctcagaaggtgttcatctttagcggaacgttcaggaagaacttggatccctacgaacaatggagtgatcaagaaatatggaaagtggcagatgaggtaggcttgcgcagtgtcattgaacaattcccagggaaactcgactttgtactggtggacggcggttgcgtcttgtcacacgggcacaaacagttgatgtgtttggcccgcagtgttttgtctaaggcgaagattctgttgctcgacgaaccgagtgctcatcttgatcccgtcacctaccaaatcatcagaaggacgttgaagcaagctttcgccgactgcactgtaatcctttgtgagcataggatcgaagcaatgctcgagtgccaacagttcttggttatagaggagaataaggttcggcaatacgactcaatacagaaactgcttaatgagcggtcactctttcgacaagctatctctcctagtgacagggtaaagctttttcctcatcggaattccagcaagtgtaagagtaaaccacagatcgccgcccttaaagaggagaccgaagaagaggtgcaggatacgagactttag

SEQ ID NO: 28 - RNA, 4688 nt, Artificial Sequence; identical to SEQ ID NO: 6
  Synthetic polynucleotide

SEQ ID NO: 29 - RNA, 4688 nt, Artificial Sequence
  Synthetic polynucleotide
ggacagaucgccuggagacgccauccacgcuguuuugaccuccauagaagacaccgggaccgauccagccuccgcggccgggaacggugcauuggaacgcggauuccccgugccaagagugacucaccguccuugacacgaugcagcgguccccgcucgaaaaggccagugucguguccaaacucuucuucucauggacucggccuauccuuagaaagggguaucggcagaggcuugaguugucugacaucuaccagauccccucgguagauucggcggauaaccucucggagaagcucgaacgggaaugggaccgcgaacucgcgucuaagaaaaacccgaagcucaucaacgcacugagaaggugcuucuucuggcgguucauguucuacgguaucuucuuguaucucggggaggucacaaaagcaguccaaccccuguuguugggucgcauuaucgccucguacgaccccgauaacaaagaagaacggagcaucgcgaucuaccucgggaucggacuguguuugcuuuucaucgucagaacacuuuuguugcauccagcaaucuucggccuccaucacaucgguaugcagaugcgaaucgcuauguuuagcuugaucuacaaaaagacacugaaacucucgucgcggguguuggauaagauuuccaucggucaguuggugucccugcuuaguaauaaccucaacaaauucgaugagggacuggcgcuggcacauuucguguggauugccccguugcaagucgcccuuuugaugggccuuauuugggagcuguugcaggcaucugccuuuuguggccugggauuucugauuguguuggcauuguuucaggcugggcuugggcggaugaugaugaaguaucgcgaccagagagcggguaaaaucucggaaagacucgucaucacuucggaaaugaucgaaaacauccagucggucaaagccuauugcugggaagaagcuauggagaagaugauugaaaaccuccgccaaacugagcugaaacugacccgcaaggcggcguauguccgguauuucaauucgucagcguucuucuuuuccggguucuucguugucuuucucucgguuuugccuuaugccuugauuaaggggauuauccuccgcaagauuuucaccacgauuucguucugcauuguauugcgcauggcagugacacggcaauuuccgugggccgugcagacaugguaugacucgcuuggagcgaucaacaaaauccaagacuucuugcaaaagcaagaguacaagacccuggaguacaaucuuacuacuacggagguaguaauggagaaugugacggcuuuuugggaagaggguuuuggagaacuguuugagaaagcaaagcagaauaacaacaaccgcaagaccucaaauggggacgauucccuguuuuucucgaacuucucccugcucggaacacccguguugaaggacaucaauuucaagauugagaggggacagcuucucgcgguagcgggaagcacuggugcgggaaaaacuagccucuugauggugauuaugggggagcuugagcccagcgaggggaagauuaaacacuccgggcguaucucauucuguagccaguuuucauggaucaugcccggaaccauuaaagagaacaucauuuucggaguauccuaugaugaguaccgauacagaucggucauuaaggcgugccaguuggaagaggacauuucuaaguucgccgagaaggauaacaucgucuugggagaaggggguauuacauugucgggagggcagcgagcgcggaucagccucgcgagagcgguauacaaagaugcagauuuguaucugcuugauucaccguuuggauaccucgacguauugacagaaaaagaaaucuucgagucgugcguguguaaacuuauggcuaauaagacgagaauccuggugacaucaaaaauggaacaccuuaagaaggcggacaagauccugauccuccacgaaggaucguccuacuuuuacggcacuuucucagaguugcaaaacuugcagccggacuucucaagcaaacucauggggugugacucauucgaccaguucagcgcggaacggcggaacucgaucuugacggaaacgcugcaccgauucucgcuugagggugaugccccgguaucguggaccgagacaaagaagcagucguuuaagcagacaggagaauuuggugagaaaagaaagaacaguaucuugaauccuauuaacucaauucgcaaguucucaaucguccagaaaacuccacugcagaugaauggaauugaagaggauucggacgaaccccuggagcgcaggcuuagccucgugccggauucagagcaaggggaggccauucuuccccggauuucggugauuucaaccggaccuacacuucaggcgaggcgaaggcaauccgugcucaaccucaugacgcauucgguaaaccaggggcaaaacauucaccgcaaaacgacggccucaacgagaaaagugucacuugcaccccaggcgaauuugacugaacucgacaucuacagccguaggcuuucgcaagaaaccggacuugagaucagcgaagaaaucaaugaagaagauuugaaagaguguuucuuugaugacauggaaucaaucccagcggugacaacguggaacacauacuugcguuacaucacggugcacaaguccuugauuuucguccucaucuggugucucgugaucuuucucgcugaggucgcagcgucacuugugguccucuggcugcuugguaauacgcccuugcaagacaaaggcaauucuacacacucaagaaacaauuccuaugccgugauuaucacuucuacaagcucguauuacguguuuuacaucuacguaggaguggccgacacucugcucgcgauggguuucuuccgaggacucccacucguucacacgcuuaucacugucuccaagauucuccaccauaagaugcuucauagcguacugcaggcucccauguccaccuugaauacgcucaaggcgggagguauuuugaaucgcuucucaaaagauauugcaauuuuggaugaccuucugccccugacgaucuucgacuucauccaguuguugcugaucgugauuggggcuauugcaguagucgcuguccuccagccuuacauuuuugucgcgaccguuccggugaucguggcguuuaucaugcugcgggccuauuucuugcagacgucacagcagcuuaagcaacuggagucugaagggaggucgccuaucuuuacgcaucuugugaccaguuugaagggauuguggacguugcgcgccuuuggcaggcagcccuacuuugaaacacuguuccacaaagcgcugaaucuccauacggcaaauugguuuuuguauuugaguacccuccgaugguuucagaugcgcauugagaugauuuuugugaucuucuuuaucgcggugacuuuuaucuccaucuugaccacgggagagggcgagggacgggucgguauuauccugacacucgccaugaacauuaugagcacuuugcagugggcagugaacagcucgauugauguggauagccugaugagguccguuucgagggucuuuaaguucaucgacaugccgacggagggaaagcccacaaaaaguacgaaacccuauaagaaugggcaauugaguaagguaaugaucaucgagaacagucacgugaagaaggaugacaucuggccuagcgggggucagaugaccgugaaggaccugacggcaaaauacaccgagggagggaacgcaauccuugaaaacaucucguucagcauuagccccggucagcgugugggguugcucgggaggaccgggucaggaaaaucgacguugcugucggccuucuugagacuucugaauacagagggugagauccagaucgacggcguuucgugggauagcaucaccuugcagcaguggcggaaagcguuuggaguaaucccccaaaaggucuuuaucuuuagcggaaccuuccgaaagaaucucgauccuuaugaacaguggucagaucaagagauuuggaaagucgcggacgagguuggccuucggaguguaaucgagcaguuuccgggaaaacucgacuuuguccuuguagaugggggaugcguccugucgcaugggcacaagcagcucaugugccuggcgcgauccguccucucuaaagcgaaaauucuucucuuggaugaaccuucggcccaucuggacccgguaacguaucagaucaucagaaggacacuuaagcaggcguuugccgacugcacggugauucucugugagcaucguaucgaggccaugcucgaaugccagcaauuucuugucaucgaagagaauaagguccgccaguacgacuccauccagaagcugcuuaaugagagaucauuguuccggcaggcgauuucaccauccgauagggugaaacuuuuuccacacagaaauucgucgaagugcaaguccaaaccgcagaucgcggccuugaaagaagagacugaagaagaaguucaagacacgcgucuuuaacggguggcaucccugugaccccuccccagugccucuccuggcccuggaaguugccacuccagugcccaccagccuuguccuaauaaaauuaaguugcaucaagcu

SEQ ID NO: 30 - RNA, 4688 nt, Artificial Sequence
  Synthetic polynucleotide
ggacagaucgccuggagacgccauccacgcuguuuugaccuccauagaagacaccgggaccgauccagccuccgcggccgggaacggugcauuggaacgcggauuccccgugccaagagugacucaccguccuugacacgaugcagaggagcccacuggagaaagccuccguggugaguaaacucuuuuuuaguuggaccagacccauccugcgaaaaggauacaggcagcgccucgaguugucugauaucuaccagauuccuucuguggacucagcugacaauuugagugagaagcuggagcgggagugggauagagagcuggcgagcaaaaaaaaccccaagcuuaucaaugcucugcgccgcugcuuuuucuggagguucauguuuuaugggaucuuccuguaccugggggaggucaccaaagcuguucagccgcuccuucuuggccgcaucaucgccagcuaugacccugauaauaaagaagaaaggucuauugcuauuuaucugggaauuggccucugcuugcucuucaucguccgcacccuucugcugcacccugccauuuuuggccuucaccacaucggcaugcaaaugagaauugccauguucucccucauuuacaaaaagacccugaaacuuuccucaagaguguuagauaaaauauccauuggucagcuggucagccugcuguccaacaaucuuaacaaauuugaugaaggcuuggcgcuggcccacuucguguggauugcaccucugcagguggcccuguugaugggacuuauaugggagcugcuucaagccucugcuuucugugggcugggcuuuuugauuguacuggcacuuuuucaggcugggcucggaagaaugaugaugaaauacagagaucagcgggccgggaagauuucagagcgacuugugaucaccagugaaaugauugaaaauauucagagcgugaaagccuacugcugggaagaagccauggagaagaugauugagaaccugaggcagacagagcucaagcucacucggaaggcugcuuauguucgcuauuucaacagcagcgccuucuucuucaguggcuucuuuguugucuuccugucuguucugccauaugcacugauaaaaggcauuauuuuacgaaagaucuucaccaccaucaguuuuugcaucguucucaggauggccgucacaagacaguuccccugggcugugcagaccugguacgauuccuugggggccaucaacaagauucaagauuucuugcaaaaacaagaauauaaaacuuuagaauacaaccucaccaccacugaaguggucauggaaaaugugacagccuuuugggaggaggguuuuggagaauuguucgagaaggcaaagcagaauaacaacaacaggaagacgagcaauggggacgacucucucuucuucagcaacuuuucacugcucgggaccccuguguugaaagauauaaacuucaagaucgagaggggccagcucuuggcuguggcaggcuccacuggagcugguaaaacaucucuucucauggugaucaugggggaacuggagccuuccgaaggaaaaaucaagcacagugggagaaucucauucugcagccaguuuuccuggaucaugcccggcaccauuaaggaaaacaucauauuuggaguguccuaugaugaguaccgcuaccggucagucaucaaagccugucaguuggaggaggacaucuccaaguuugcagagaaagacaacauugugcuuggagagggggguaucacucuuucuggaggacaaagagccaggaucucuuuggcccgggcagucuacaaggaugcagaccucuacuuguuggacagucccuucggcuaccucgacgugcugacugaaaaagaaauuuuugaaagcugugugugcaaacugauggcaaacaagaccaggauucuugucaccagcaagauggaacaucugaagaaagcggacaaaauucugauucugcaugaagggagcuccuacuucuauggaacauuuagcgagcuucagaaccuacagccagacuucuccuccaaauuaaugggcugugacuccuucgaccaguucucugcagaaagaagaaacucuauacucacagagacccuccaccgcuucucccuugagggagaugccccaguuucuuggacagaaaccaagaagcaguccuuuaagcagacuggcgaguuuggugaaaagaggaaaaauucaauucucaauccaauuaacaguauucgcaaguucagcauuguccagaagacaccccuccagaugaauggcaucgaagaagauagugacgagccgcuggagagacggcugagucuggugccagauucagaacagggggaggccauccugccccggaucagcgucauuuccacaggccccacauuacaagcacggcgccggcagaguguuuuaaaucucaugacccauucagugaaccagggccaaaauauccacaggaagacuacagcuucuacccggaaagugucucuggccccucaggccaaucugaccgagcuggacaucuacagcaggaggcucucccaggaaacagggcuggaaauaucugaagagauuaaugaagaggaucuuaaagagugcuucuuugaugacauggagagcauccccgcggugaccacauggaacaccuaccuuagauauauuacuguccacaagagccucauauuuguccucaucuggugccugguuauuuuccucgcugagguggcggccagucuuguugugcucuggcugcugggcaacacuccucuccaggacaagggcaauaguacucacagcagaaauaauucuuaugccgucaucauuacaagcaccuccagcuacuacguguucuacaucuaugugggcguggcugacacccuccuggccauggguuucuuccggggccugccuuuggugcacacccucaucacagugucaaaaauucugcaccauaaaaugcuucauucuguccugcaggcacccaugagcacuuugaacacauugaaggcuggcggcauccucaacagauuuucuaaagauauugcuauccuggaugaucuccucccccugacaaucuuugacuuuauccagcuucugcugaucgugauuggagccauagcagugguugcuguccugcagcccuacauuuuuguggccaccgugcccgugauuguugccuuuauuaugcucagagcuuacuuccugcaaacuucucaacagcucaaacagcuagaaucugagggccggagccccauuuuuacccaccuggugacuucccugaagggacuguggacucugagagcauucgggcgacagccuuacuuugagacacuguuccacaaggcccugaacuugcacacugccaacugguuucuuuaccugagcacacuccgcugguuccagaugcggauagagaugaucuucgucaucuuuuuuauagcuguaaccuucauuucuauccuuacaacaggagaaggagagggcagggugggaaucauccucacgcuggcuaugaacauaauguccaccuugcagugggccgugaauuccaguauagauguggauucucuaaugaggagugucucccggguguuuaaauucauugauaugccuacugaggggaaacccaccaagucaacaaaaccuuauaagaauggacagcugagcaaggugaugauaauugagaacagccacgugaagaaggaugacauuuggcccagcgggggccagaugacugugaaggaccugacggccaaguacaccgaagguggaaaugccauuuuggaaaacaucagcuucucaaucucuccugggcagagaguuggauugcugggucgcacgggcagcggcaaaucaacccugcucagugccuuccuucggcuccugaauacagaaggcgaaauccaaauugacggggugagcugggacagcaucacccugcagcaguggagaaaagcauuuggggucauuccacagaaaguuuucaucuucucuggcacuuucagaaagaaccuggaccccuaugagcaguggagcgaccaggagaucuggaagguugcagaugaaguuggccugcggagugugauagaacaauuuccuggcaagcuggauuuugugcugguagauggaggcugcgugcugucccacggccacaaacagcugaugugccucgcccgcuccguucuuucaaaggccaaaaucuugcuuuuggaugagcccagugcucaccuugacccagugaccuaucagauaauccgcaggaccuuaaagcaagcuuuugccgacugcaccgucauacugugugagcaccggauugaagcaaugcuggaaugccagcaguuucuggugaucgaggagaauaagguccggcaguacgacagcauccagaaguuguugaaugagcgcagccuuuuccgccaggccaucuccccaucugacagagucaagcuguuuccacauaggaacuccucuaagugcaaguccaagccccagaucgcugcccucaaggaggaaacugaggaagaggugcaggauacccgccugugacggguggcaucccugugaccccuccccagugccucuccuggcccuggaaguugccacuccagugcccaccagccuuguccuaauaaaauuaaguugcaucaagcu